European Patent Application EP 4 545 563 A1, published April 30, 2025. Title: ANTIBODY TARGETING ITGA2 AND ANTIBODY-DRUG CONJUGATE COMPRISING THE SAME. Applicant: Foreseen Technology (Beijing) Co., Ltd. The sequence listing filed with the application follows.

SEQUENCE LISTING (219 sequences)

SEQ ID NO: 1 - DNA, 642 bp, synthetic construct
  source 1..642: mol_type = other DNA
gacatccagttgacccagtctccatcctccctgtctgcatctgtaggagacagagtcaccatcacttgccgggcaagtcagagcattatcagctatttaaattggtatcagcagaaaccagggaaagcccctaagctcctgatctatgctgcatccagtttgcaaagtggggtcccatcaaggttcagtggcagtggatctgggacagatttcactctcaccatcagcagtctgcaacctgaagattttgcaacttactactgtcaacagagttacagtacccctgacacttttggccaggggaccaagctggagatcaaaaggaccgtggctgcccccagcgtgttcatcttccctcctagcgacgagcagctgaagagcggcaccgctagcgtggtgtgtctgctgaataacttctatcccagggaggccaaggtgcagtggaaggtggataacgccctgcagagcggcaactcccaggagtccgtgaccgagcaggactccaaggacagcacctactccctgagctccaccctgaccctgtccaaggctgattatgagaagcacaaggtgtatgcttgcgaggtgacacaccagggcctgtccagccctgtgaccaagagcttcaaccggggcgagtgc

SEQ ID NO: 2 - DNA, 642 bp, synthetic construct
  source 1..642: mol_type = other DNA
gaaattgtgttgacacagtctccagccaccctgtctttgtctccaggggaaagagccaccctctcctgcagggccagtcagagtgttagcagcaacttaggctggtaccaacagaaacctggccaggctcccagcctcctcatctatggtgcatccaacagggccactggcatcccagccaggttcagtggcagtgggtctgggacagacttcactctcaccatcagcagcctagagcctgaagattttgcagtttattactgtcagcagcgtgacacctggcccctcactttcggcggagggaccaaggtggagatcaaaaggaccgtggctgcccccagcgtgttcatcttccctcctagcgacgagcagctgaagagcggcaccgctagcgtggtgtgtctgctgaataacttctatcccagggaggccaaggtgcagtggaaggtggataacgccctgcagagcggcaactcccaggagtccgtgaccgagcaggactccaaggacagcacctactccctgagctccaccctgaccctgtccaaggctgattatgagaagcacaaggtgtatgcttgcgaggtgacacaccagggcctgtccagccctgtgaccaagagcttcaaccggggcgagtgc

SEQ ID NO: 3 - DNA, 642 bp, synthetic construct
  source 1..642: mol_type = other DNA
gaaattgtgttgacacagtctccagccaccctgcctttgtctccgggggaaagagccaccctctcctgcagggccagtcagagtgttggcttctacttagcctggtaccaacagaaacctggccagcctcccagactcctcttctatgatgcatccaagagggccactggcatcccagccaggttcagcgccagtgggtctgggacagacttcactctcaccatcagcggcctagagcctgaagattttgcagtttattactgtcagcaccgcataagctggcctctgacgttcggccaagggaccaaggtggaagtgaagaggaccgtggctgcccccagcgtgttcatcttccctcctagcgacgagcagctgaagagcggcaccgctagcgtggtgtgtctgctgaataacttctatcccagggaggccaaggtgcagtggaaggtggataacgccctgcagagcggcaactcccaggagtccgtgaccgagcaggactccaaggacagcacctactccctgagctccaccctgaccctgtccaaggctgattatgagaagcacaaggtgtatgcttgcgaggtgacacaccagggcctgtccagccctgtgaccaagagcttcaaccggggcgagtgc

SEQ ID NO: 4 - DNA, 642 bp, synthetic construct
  source 1..642: mol_type = other DNA
gaaattgtgttgacacagtctccagccaccctgtctttgtctccaggggaaagagccaccctctcctgcagggccagtcagagtgttagtacttacttagcctggtaccaacagaaacctggccaggctcccaggctcctcatctatgacacatccatcagggccactggcatcccagccaggttcagtggcagtgggtctgggacagacttcactctcaccatcagcagcctagagcctgaagattttgcagtttattactgtcagcagcgtagcaactggccgctcactttcggcggagggaccaaggtggagatcaaaaggaccgtggctgcccccagcgtgttcatcttccctcctagcgacgagcagctgaagagcggcaccgctagcgtggtgtgtctgctgaataacttctatcccagggaggccaaggtgcagtggaaggtggataacgccctgcagagcggcaactcccaggagtccgtgaccgagcaggactccaaggacagcacctactccctgagctccaccctgaccctgtccaaggctgattatgagaagcacaaggtgtatgcttgcgaggtgacacaccagggcctgtccagccctgtgaccaagagcttcaaccggggcgagtgc

SEQ ID NO: 5 - DNA, 642 bp, synthetic construct
  source 1..642: mol_type = other DNA
gaaattgtgttgacacagtctccagccatcctgtctttgtctccaggggaaagagccaccctctcctgcagggccagtcagagtgttagcgagtacttagcctggtaccaacaaaaacctggccaggctcccaggctcctcatctatgatatatctaacagggccactggcatcccagccaggttcagtggcagtgggtctgagacagacttcactctcaccatcagcagcctagagcctgaagattttgcagtttattactgtcaacaacgtcgcacctggcctctcactttcggccctgggaccaaagtggacatcaaaaggaccgtggctgcccccagcgtgttcatcttccctcctagcgacgagcagctgaagagcggcaccgctagcgtggtgtgtctgctgaataacttctatcccagggaggccaaggtgcagtggaaggtggataacgccctgcagagcggcaactcccaggagtccgtgaccgagcaggactccaaggacagcacctactccctgagctccaccctgaccctgtccaaggctgattatgagaagcacaaggtgtatgcttgcgaggtgacacaccagggcctgtccagccctgtgaccaagagcttcaaccggggcgagtgc

SEQ ID NO: 6 - DNA, 642 bp, synthetic construct
  source 1..642: mol_type = other DNA
aacatccagttgacccagtctccacccttcctgtctgcatctgtaggagacagagtcaccatcacttgccgggccagccaggacattagcagttttttagcctggtatcagcaaaaaccagggaaagcccctaacctcctgatccatgctgcaaccactctgcaaagtggggtcccatcaaggttcagcggcagtggatctgggacggagttcactctcacaatcagcagcctgcggccagaagattttgccacttactactgtcaacaacttcatacttacccgatcaccttcggccaagggacacgactggagattaaacgaactgtggctgcaccatccgtgttcatcttccctcctagcgacgagcagctgaagagcggcaccgctagcgtggtgtgtctgctgaataacttctatcccagggaggccaaggtgcagtggaaggtggataacgccctgcagagcggcaactcccaggagtccgtgaccgagcaggactccaaggacagcacctactccctgagctccaccctgaccctgtccaaggctgattatgagaagcacaaggtgtatgcttgcgaggtgacacaccagggcctgtccagccctgtgaccaagagcttcaaccggggcgagtgc

SEQ ID NO: 7 - DNA, 639 bp, synthetic construct
  source 1..639: mol_type = other DNA
aacatccagatgacccagtctccaccctccctgtctgcatctgtgggagacagagtcgccatcacttgccgggcgagtcaggacattagcaattccttagcctggtatcagcagaagtcagggcaaccccctaaactcctgctctatgatgtgtcgaaattggaaaggggggtcccatccaggttcagtggcagtggatctcggacggattacactctcaccatcagcagcctgcagcctgaagattttgcaacttattactgtcaacagtattctagtgaccccacttttggacaggggagtaagctggagttcaaacgaactgtggctgcaccatccgtgttcatcttccctcctagcgacgagcagctgaagagcggcaccgctagcgtggtgtgtctgctgaataacttctatcccagggaggccaaggtgcagtggaaggtggataacgccctgcagagcggcaactcccaggagtccgtgaccgagcaggactccaaggacagcacctactccctgagctccaccctgaccctgtccaaggctgattatgagaagcacaaggtgtatgcttgcgaggtgacacaccagggcctgtccagccctgtgaccaagagcttcaaccggggcgagtgc

SEQ ID NO: 8 - DNA, 642 bp, synthetic construct
  source 1..642: mol_type = other DNA
gacatccagatgatccagtctccttcttccgtgtctgcttctgtgggagacagagtcaccatcacttgtcgggcgagtcagggtatcagcaactcgttagcctggtatcagcacaaaccaggtacaacccctaagctcctgatctatgctgcatccagtttgcaaggtggggtcccatccaggttcagcggcagttcatctgagacagatttcactctcaccatcagcagccttcagcctgaagattttgcaacttactactgtcagcaggccaacagtttcccgatcaccttcggccaggggacacgactggatattaaacgaactgtggctgcaccatccgtgttcatcttccctcctagcgacgagcagctgaagagcggcaccgctagcgtggtgtgtctgctgaataacttctatcccagggaggccaaggtgcagtggaaggtggataacgccctgcagagcggcaactcccaggagtccgtgaccgagcaggactccaaggacagcacctactccctgagctccaccctgaccctgtccaaggctgattatgagaagcacaaggtgtatgcttgcgaggtgacacaccagggcctgtccagccctgtgaccaagagcttcaaccggggcgagtgc

SEQ ID NO: 9 - DNA, 645 bp, synthetic construct
  source 1..645: mol_type = other DNA
gaaattgtgttgacacagtctccagccactctgtctttgtctccaggggaaagagccaccctctcctgcagggccagtcagagtgttagcagctacttagcctggtaccaacaaaaacctggccaggctcccagactcctcatctatgatgcatccaacagggccactggcatcccagccaggttcagtggcagtgggtctgggacagacttcactctcaccatcagcagcctagagcctgaagattttgcagtttattactgtcagcagcgtaccaactggcttatgtacacttttggccaggggaccaagctggagatcaaacgaactgtggctgcaccatccgtgttcatcttccctcctagcgacgagcagctgaagagcggcaccgctagcgtggtgtgtctgctgaataacttctatcccagggaggccaaggtgcagtggaaggtggataacgccctgcagagcggcaactcccaggagtccgtgaccgagcaggactccaaggacagcacctactccctgagctccaccctgaccctgtccaaggctgattatgagaagcacaaggtgtatgcttgcgaggtgacacaccagggcctgtccagccctgtgaccaagagcttcaaccggggcgagtgc

SEQ ID NO: 10 - DNA, 642 bp, synthetic construct
  source 1..642: mol_type = other DNA
gaaattgtgttgacacagtctccagccaccctgtctttgtctccaggggaaagagccaccctctcctgcagggccagtcagagtgttagcagctacttagcctggtaccaacagaaacctggccaggctcccaggctcctcatctatgatgcatccaacagggccactggcatcccagccaggttcagtggcagtgggtctgggacagacttcactctcaccatcagcagcctagagcctgaagattttgcagtttattactgtcagcagcgtagcaactggcccctcactttcggcggagggaccaaggtggagatcaaacgaactgtggctgcaccatccgtgttcatcttccctcctagcgacgagcagctgaagagcggcaccgctagcgtggtgtgtctgctgaataacttctatcccagggaggccaaggtgcagtggaaggtggataacgccctgcagagcggcaactcccaggagtccgtgaccgagcaggactccaaggacagcacctactccctgagctccaccctgaccctgtccaaggctgattatgagaagcacaaggtgtatgcttgcgaggtgacacaccagggcctgtccagccctgtgaccaagagcttcaaccggggcgagtgc

SEQ ID NO: 11 - DNA, 639 bp, synthetic construct
  source 1..639: mol_type = other DNA
aacatccagatgacccagtctccatcctccctgtctgcatctgtaggagacagagtcaccatcacttgccgggcaagtcagagcattagcagctatttaaattggtatcagcagaaaccagggaaagcccctaagctcctgatctatgctgcatccagtttgcaaagtggggtcccatcaaggttcagtggcagtggatctgggacagatttcactctcaccatcagcagtctgcaacctgaagattttgcatcttactactgtcaacagagttacagttcgtgggcgttcggccaagggaccaaggtggaaatcaaacgaactgtggctgcaccatccgtgttcatcttccctcctagcgacgagcagctgaagagcggcaccgctagcgtggtgtgtctgctgaataacttctatcccagggaggccaaggtgcagtggaaggtggataacgccctgcagagcggcaactcccaggagtccgtgaccgagcaggactccaaggacagcacctactccctgagctccaccctgaccctgtccaaggctgattatgagaagcacaaggtgtatgcttgcgaggtgacacaccagggcctgtccagccctgtgaccaagagcttcaaccggggcgagtgc

SEQ ID NO: 12 - DNA, 642 bp, synthetic construct
  source 1..642: mol_type = other DNA
aacatccagttgacccagtctccatcttccgtgtctgcatctgtaggagacagagtcaccatcacttgtcgggcgagtcagggttttagtaggtggttagcctggtatcagcagaaaccagggaaagcccctaagctcctgatctatggtgcatccagtttgcaaagtggggtcccatcaagattcagcggcagtggatctgggacagatttcactctcaccatcagcagcctgcagcctgaagattttgcaacttactattgtcaacaggctaacagtttccctctcactttcggcggagggaccaagctggagatcaaacgaactgtggctgcaccatccgtgttcatcttccctcctagcgacgagcagctgaagagcggcaccgctagcgtggtgtgtctgctgaataacttctatcccagggaggccaaggtgcagtggaaggtggataacgccctgcagagcggcaactcccaggagtccgtgaccgagcaggactccaaggacagcacctactccctgagctccaccctgaccctgtccaaggctgattatgagaagcacaaggtgtatgcttgcgaggtgacacaccagggcctgtccagccctgtgaccaagagcttcaaccggggcgagtgc

SEQ ID NO: 13 - DNA, 642 bp, synthetic construct
  source 1..642: mol_type = other DNA
aacatccagttgacccagtctccatcctccctgtctgcatctgtaggagacagagtcaccatcacttgccgggcaagtcagagcattagcagctatttaaattggtatcagcagaaaccagggaaagcccctaagctcctgatctatgctgcatccagtttgcaaagtggggtcccatcaaggttcagtggcagtggatctgggacagatttcactctcaccatcagcagtctgcaacctgaagattttgcaacttactactgtcaacagagttacagtaccccagacactttcggccctgggaccaaagtggatatcaaacgaactgtggctgcaccatccgtgttcatcttccctcctagcgacgagcagctgaagagcggcaccgctagcgtggtgtgtctgctgaataacttctatcccagggaggccaaggtgcagtggaaggtggataacgccctgcagagcggcaactcccaggagtccgtgaccgagcaggactccaaggacagcacctactccctgagctccaccctgaccctgtccaaggctgattatgagaagcacaaggtgtatgcttgcgaggtgacacaccagggcctgtccagccctgtgaccaagagcttcaaccggggcgagtgc

SEQ ID NO: 14 - DNA, 648 bp, synthetic construct
  source 1..648: mol_type = other DNA
cagtctgccctgactcagcctgcctccgtgtctgggtctcctggacagtcgatcaccatctcctgcactggaaccagcagtgacgttggtggttataactatgtctcctggtaccaacaacacccaggcaaagcccccaaactcatgatttatgatgtcagtaatcggccctcaggggtttctaatcgcttctctggctccaagtctggcaacacggcctccctgaccatctctgggctccaggctgaggacgaggctgattattattgcagctcatttacaaccatcactacgagggtgttcggcggagggaccaagctgaccgtcctaggtcagcccaaggctgccccctcggtgacactgttccctccatcctctgaggaactgcaggccaacaaggctaccctcgtgtgcctgatctccgacttttaccctggcgctgtgaccgtggcctggaaggctgatagttctcctgtgaaggccggcgtggaaaccaccacaccttccaagcagtccaacaacaaatacgccgcctcctcctacctgtctctgacccctgaacagtggaagtcccaccggtcctacagctgccaagtgacccatgagggctccaccgtggaaaagaccgtggctcctaccgagtgctct

SEQ ID NO: 15 - DNA, 648 bp, synthetic construct
  source 1..648: mol_type = other DNA
cagtctgccctgactcagcctgcctccgtgtctgggtctcctggacagtcgatcaccatctcctgcagtggaaccagcagtgacattggtcgttataactatgtctcctggtaccaacaacacccaggcaaagcccccaaactcctgatttttgatgtcagtaatcggccctcaggggtttctaatcgtttctctggctccaagtctggcaacacggcctccctgaccatctctgggctccaggctgaggacgaggctgattattactgcagctcatatacaagcaccgtcccttatgtcttcggaactgggacgcgggtcgccgtccaaggtcagcccaaggctgccccctcggtgacactgttccctccatcctctgaggaactgcaggccaacaaggctaccctcgtgtgcctgatctccgacttttaccctggcgctgtgaccgtggcctggaaggctgatagttctcctgtgaaggccggcgtggaaaccaccacaccttccaagcagtccaacaacaaatacgccgcctcctcctacctgtctctgacccctgaacagtggaagtcccaccggtcctacagctgccaagtgacccatgagggctccaccgtggaaaagaccgtggctcctaccgagtgctct

SEQ ID NO: 16 - DNA, 648 bp, synthetic construct
  source 1..648: mol_type = other DNA
gaaattgtattgacacagtctccagccaccctgtctttgtctccaggggaaagagccaccctctcctgccaggccagtcagacttttagcgattacttagcctggtaccaacagaaacctggccaggctcccaggctcctcatctatgatgcatccaccagggccactggcatcccagccaggttcagtggcagtgggtctgggacagacttcactctcaccatcagcagcctagagcctgaagattttgcagtttattactgtcagcagcgtagccactggcctccagggtacacttttggccaagggaccagggtggagatcaaacgaactgtggctgcaccatccgtgttcatcttccctcctagcgacgagcagctgaagagcggcaccgctagcgtggtgtgtctgctgaataacttctatcccagggaggccaaggtgcagtggaaggtggataacgccctgcagagcggcaactcccaggagtccgtgaccgagcaggactccaaggacagcacctactccctgagctccaccctgaccctgtccaaggctgattatgagaagcacaaggtgtatgcttgcgaggtgacacaccagggcctgtccagccctgtgaccaagagcttcaaccggggcgagtgc

SEQ ID NO: 17 - DNA, 642 bp, synthetic construct
  source 1..642: mol_type = other DNA
gaaattgtgttgacacagtctccagccaccctgtctttgtctccaggggaaagagccaccctctcctgcagggccagtcagagtgtttacagttctttagcctggtaccaacagaaacctggccaggctcccaagctcctcatctatgatgcatccaacagggccactggcgtcccagccaggttcagtggcagtgggtctgggacagacttcactctcaccatcagcagcctagagcctgaggattttgcactttattactgtcagcaccgtcagcattggcctctcactttcggcggagggaccaaggtggagatcaaacgaactgtggctgcaccatccgtgttcatcttccctcctagcgacgagcagctgaagagcggcaccgctagcgtggtgtgtctgctgaataacttctatcccagggaggccaaggtgcagtggaaggtggataacgccctgcagagcggcaactcccaggagtccgtgaccgagcaggactccaaggacagcacctactccctgagctccaccctgaccctgtccaaggctgattatgagaagcacaaggtgtatgcttgcgaggtgacacaccagggcctgtccagccctgtgaccaagagcttcaaccggggcgagtgc

SEQ ID NO: 18 - DNA, 642 bp, synthetic construct
  source 1..642: mol_type = other DNA
gaaattgtgatgacgcagtctccagtcaccctgtctgtctctccaggggactcagccaccctctcctgcagggccagtcagagtgttgataaaaacttagcctggtaccagcagaaaactggccaggctcccaggctcctcatctatggtgcagccaccagggccactggtatcccagccaggttcagtggcagtgggtctgggacagaattcactctcaccatcagcagcctgcggtctgaagattttgcagtttattactgtcagcagtatagaaactggccttggacgttcggcctagggaccaaggtggagatcaaacgaactgtggctgcaccatccgtgttcatcttccctcctagcgacgagcagctgaagagcggcaccgctagcgtggtgtgtctgctgaataacttctatcccagggaggccaaggtgcagtggaaggtggataacgccctgcagagcggcaactcccaggagtccgtgaccgagcaggactccaaggacagcacctactccctgagctccaccctgaccctgtccaaggctgattatgagaagcacaaggtgtatgcttgcgaggtgacacaccagggcctgtccagccctgtgaccaagagcttcaaccggggcgagtgc

SEQ ID NO: 19 - DNA, 1356 bp, synthetic construct
  source 1..1356: mol_type = other DNA
caggtgcagctggtgcaatctggggctgaggtgaagaagcctggggcctcagtgaaggtttcctgcaaggcatctggatacaccttcaccagctactatatgcactgggtgcgacaggcccctggacaagggcttgagtggatgggaataatcaaccctagtggtggtagcacaagctacgcacagaagttccagggcagagtcaccatgaccagggacacgtccacgagcacagtctacatggagctgagcagcctgagatctgaggacacggccgtgtattactgtgcgagagatattagtgggagctaccaaactgatgcttttgatatctggggccaagggacaatggtcaccgtctcatcagcttccaccaagggcccctccgtgttccccctggctccctcttccaagagcaccagcggcggcaccgctgctctgggatgtctggtgaaggactacttccctgagcctgtgaccgtgtcctggaattccggcgccctgacctccggcgtgcacacattccctgctgtgctgcagtcctccggcctgtatagcctgtcctccgtggtgacagtgcctagctccagcctgggcacccagacctatatctgcaacgtgaaccacaagcctagcaataccaaggtggacaagaaggtggagcctaagagctgcgacaagacccacacctgtcctccatgtcctgctccagaactgctcggcggaccttccgtgttcctgtttcctccaaagcctaaggacaccctgatgatcagcagaacccctgaagtgacctgcgtggtggtggatgtgtcccacgaggatcccgaagtgaagttcaattggtacgtggacggcgtggaagtgcacaacgccaagaccaagcctagagaggaacagtacaacagcacctacagagtggtgtccgtgctgaccgtgctgcaccaggattggctgaacggcaaagagtacaagtgcaaggtgtccaacaaggccctgcctgctcctatcgagaaaaccatcagcaaggccaagggccagcctagggaaccccaggtttacacactgcctccaagcagggacgagctgaccaagaatcaggtgtccctgacctgcctggtcaagggcttctacccttccgatatcgccgtggaatgggagagcaatggccagcctgagaacaactacaagacaacccctcctgtgctggacagcgacggctcattcttcctgtacagcaagctgacagtggacaagagcagatggcagcagggcaacgtgttcagctgcagcgtgatgcacgaggccctgcacaaccactacacccagaagtccctgagcctgtctcctggcaaa

SEQ ID NO: 20 - DNA, 1353 bp, synthetic construct
  source 1..1353: mol_type = other DNA
caggtgcagctgcaggactcgggcccaggactggtgaagccttcacagaccctgtccctcacctgcactgtctctggtggctccatcagcagtggtggttactactggagctggatccgccagcacccagggaagggcctggagtggattgggtacatctattacagtgggagcacctactacaacccgtccctcaagagtcgagttaccatatcagtagacacgtctaagaaccagttctccctgaagctgagctctgtgactgccgcggacacggccgtgtattactgtgcgagagtgcctgtcccactggtgggggcttttgatatctggggccaagggacaatggtcaccgtctcatcagcttccaccaagggcccctccgtgttccccctggctccctcttccaagagcaccagcggcggcaccgctgctctgggatgtctggtgaaggactacttccctgagcctgtgaccgtgtcctggaattccggcgccctgacctccggcgtgcacacattccctgctgtgctgcagtcctccggcctgtatagcctgtcctccgtggtgacagtgcctagctccagcctgggcacccagacctatatctgcaacgtgaaccacaagcctagcaataccaaggtggacaagaaggtggagcctaagagctgcgacaagacccacacctgtcctccatgtcctgctccagaactgctcggcggaccttccgtgttcctgtttcctccaaagcctaaggacaccctgatgatcagcagaacccctgaagtgacctgcgtggtggtggatgtgtcccacgaggatcccgaagtgaagttcaattggtacgtggacggcgtggaagtgcacaacgccaagaccaagcctagagaggaacagtacaacagcacctacagagtggtgtccgtgctgaccgtgctgcaccaggattggctgaacggcaaagagtacaagtgcaaggtgtccaacaaggccctgcctgctcctatcgagaaaaccatcagcaaggccaagggccagcctagggaaccccaggtttacacactgcctccaagcagggacgagctgaccaagaatcaggtgtccctgacctgcctggtcaagggcttctacccttccgatatcgccgtggaatgggagagcaatggccagcctgagaacaactacaagacaacccctcctgtgctggacagcgacggctcattcttcctgtacagcaagctgacagtggacaagagcagatggcagcagggcaacgtgttcagctgcagcgtgatgcacgaggccctgcacaaccactacacccagaagtccctgagcctgtctcctggcaaa

SEQ ID NO: 21 - DNA, 1347 bp, synthetic construct
  source 1..1347: mol_type = other DNA
cggctgcagctgcaggagtcgggcccaggactggtgaagccttcacagaccctgtccctcacctgcactgtctctggtggctccatcagcagtggtggttactactggagctggatccgccagcacccagggaagggcctggagtggattgggtacatctattacagtgggagcacctactacaacccgtccctcaagagtcgagttaccatatcagtagacacgtctaagaaccagttctccctgaagctgagctctgtgactgccgcggacacggccgtgtattactgtgcgagagcaaccatctacggttactttgactactggggccagggaaccctggtcaccgtctcatcagcttccaccaagggcccctccgtgttccccctggctccctcttccaagagcaccagcggcggcaccgctgctctgggatgtctggtgaaggactacttccctgagcctgtgaccgtgtcctggaattccggcgccctgacctccggcgtgcacacattccctgctgtgctgcagtcctccggcctgtatagcctgtcctccgtggtgacagtgcctagctccagcctgggcacccagacctatatctgcaacgtgaaccacaagcctagcaataccaaggtggacaagaaggtggagcctaagagctgcgacaagacccacacctgtcctccatgtcctgctccagaactgctcggcggaccttccgtgttcctgtttcctccaaagcctaaggacaccctgatgatcagcagaacccctgaagtgacctgcgtggtggtggatgtgtcccacgaggatcccgaagtgaagttcaattggtacgtggacggcgtggaagtgcacaacgccaagaccaagcctagagaggaacagtacaacagcacctacagagtggtgtccgtgctgaccgtgctgcaccaggattggctgaacggcaaagagtacaagtgcaaggtgtccaacaaggccctgcctgctcctatcgagaaaaccatcagcaaggccaagggccagcctagggaaccccaggtttacacactgcctccaagcagggacgagctgaccaagaatcaggtgtccctgacctgcctggtcaagggcttctacccttccgatatcgccgtggaatgggagagcaatggccagcctgagaacaactacaagacaacccctcctgtgctggacagcgacggctcattcttcctgtacagcaagctgacagtggacaagagcagatggcagcagggcaacgtgttcagctgcagcgtgatgcacgaggccctgcacaaccactacacccagaagtccctgagcctgtctcctggcaaa

SEQ ID NO: 22 - DNA, 1350 bp, synthetic construct
  source 1..1350: mol_type = other DNA
caggtgcagctgcaggagtcgggcccaggactggtgaagccttcacagaccctgtccctcacctgcactgtctctggtggctccatcagcagtggtggttactactggagctggatccgccagcacccagggaagggcctggagtggattgggtacatctattacagtgggagcacctactacaacccgtccctcaagagtcgagttaccatatcagtagacacgtctaagaaccagttctccctgaagctgagctctgtgactgccgcggacacggccgtgtactactgtgcgagagtccgcctattgggtggtggttttgatatctggggccaagggaccacggtcaccgtctcatcagcttccaccaagggcccctccgtgttccccctggctccctcttccaagagcaccagcggcggcaccgctgctctgggatgtctggtgaaggactacttccctgagcctgtgaccgtgtcctggaattccggcgccctgacctccggcgtgcacacattccctgctgtgctgcagtcctccggcctgtatagcctgtcctccgtggtgacagtgcctagctccagcctgggcacccagacctatatctgcaacgtgaaccacaagcctagcaataccaaggtggacaagaaggtggagcctaagagctgcgacaagacccacacctgtcctccatgtcctgctccagaactgctcggcggaccttccgtgttcctgtttcctccaaagcctaaggacaccctgatgatcagcagaacccctgaagtgacctgcgtggtggtggatgtgtcccacgaggatcccgaagtgaagttcaattggtacgtggacggcgtggaagtgcacaacgccaagaccaagcctagagaggaacagtacaacagcacctacagagtggtgtccgtgctgaccgtgctgcaccaggattggctgaacggcaaagagtacaagtgcaaggtgtccaacaaggccctgcctgctcctatcgagaaaaccatcagcaaggccaagggccagcctagggaaccccaggtttacacactgcctccaagcagggacgagctgaccaagaatcaggtgtccctgacctgcctggtcaagggcttctacccttccgatatcgccgtggaatgggagagcaatggccagcctgagaacaactacaagacaacccctcctgtgctggacagcgacggctcattcttcctgtacagcaagctgacagtggacaagagcagatggcagcagggcaacgtgttcagctgcagcgtgatgcacgaggccctgcacaaccactacacccagaagtccctgagcctgtctcctggcaaa

SEQ ID NO: 23 - DNA, 1362 bp, synthetic construct
  source 1..1362: mol_type = other DNA
gaggtacaactggtggagtctgggggaggcgtggtccagcctgggaggtccctgagactctcctgtgcagcctctggattcaccttcagtagctatgctatgcactgggtccgccaggctccaggcaaggggctggagtgggtggcagttatatcatatgatggaagtaataaatactacgtagactccgtgaagggccgattcaccatctccagagacaattccaagaacacgctgtatctgcaaatgaacagcctgagagctgaggacacggctgtgtattactgtgcgagagatcgtataacgtatcttgactactactactacggtatggacgtctggggccaagggaccacggtcaccgtctcatcagcttccaccaagggcccctccgtgttccccctggctccctcttccaagagcaccagcggcggcaccgctgctctgggatgtctggtgaaggactacttccctgagcctgtgaccgtgtcctggaattccggcgccctgacctccggcgtgcacacattccctgctgtgctgcagtcctccggcctgtatagcctgtcctccgtggtgacagtgcctagctccagcctgggcacccagacctatatctgcaacgtgaaccacaagcctagcaataccaaggtggacaagaaggtggagcctaagagctgcgacaagacccacacctgtcctccatgtcctgctccagaactgctcggcggaccttccgtgttcctgtttcctccaaagcctaaggacaccctgatgatcagcagaacccctgaagtgacctgcgtggtggtggatgtgtcccacgaggatcccgaagtgaagttcaattggtacgtggacggcgtggaagtgcacaacgccaagaccaagcctagagaggaacagtacaacagcacctacagagtggtgtccgtgctgaccgtgctgcaccaggattggctgaacggcaaagagtacaagtgcaaggtgtccaacaaggccctgcctgctcctatcgagaaaaccatcagcaaggccaagggccagcctagggaaccccaggtttacacactgcctccaagcagggacgagctgaccaagaatcaggtgtccctgacctgcctggtcaagggcttctacccttccgatatcgccgtggaatgggagagcaatggccagcctgagaacaactacaagacaacccctcctgtgctggacagcgacggctcattcttcctgtacagcaagctgacagtggacaagagcagatggcagcagggcaacgtgttcagctgcagcgtgatgcacgaggccctgcacaaccactacacccagaagtccctgagcctgtctcctggcaaa

SEQ ID NO: 24 - DNA, 1350 bp, synthetic construct
  source 1..1350: mol_type = other DNA
caggtacagctgcagcagtcaggtccaggactggtgaagccctcgcagaccctctcacttacctgtgccatctccggggacagtgtctctagcgacagtgctgcttggaactggatcaggcagtccccatcgagaggccttgagtggctgggaaggacatactacaggtccaagtggtataatgattatgcagtatctgtgaaaagtcgaataaccatcaacccagacacatccaagaaccagttctccctgcagctaaattctgtgacttccgacgacacggctgtgtattactgtgcaagaggctcttgggcggctccatggttgtggggccagggaaccctggtcaccgtctcatcagcttccaccaagggcccctccgtgttccccctggctccctcttccaagagcaccagcggcggcaccgctgctctgggatgtctggtgaaggactacttccctgagcctgtgaccgtgtcctggaattccggcgccctgacctccggcgtgcacacattccctgctgtgctgcagtcctccggcctgtatagcctgtcctccgtggtgacagtgcctagctccagcctgggcacccagacctatatctgcaacgtgaaccacaagcctagcaataccaaggtggacaagaaggtggagcctaagagctgcgacaagacccacacctgtcctccatgtcctgctccagaactgctcggcggaccttccgtgttcctgtttcctccaaagcctaaggacaccctgatgatcagcagaacccctgaagtgacctgcgtggtggtggatgtgtcccacgaggatcccgaagtgaagttcaattggtacgtggacggcgtggaagtgcacaacgccaagaccaagcctagagaggaacagtacaacagcacctacagagtggtgtccgtgctgaccgtgctgcaccaggattggctgaacggcaaagagtacaagtgcaaggtgtccaacaaggccctgcctgctcctatcgagaaaaccatcagcaaggccaagggccagcctagggaaccccaggtttacacactgcctccaagcagggacgagctgaccaagaatcaggtgtccctgacctgcctggtcaagggcttctacccttccgatatcgccgtggaatgggagagcaatggccagcctgagaacaactacaagacaacccctcctgtgctggacagcgacggctcattcttcctgtacagcaagctgacagtggacaagagcagatggcagcagggcaacgtgttcagctgcagcgtgatgcacgaggccctgcacaaccactacacccagaagtccctgagcctgtctcctggcaaa

SEQ ID NO: 25 - DNA, 1341 bp, synthetic construct
  source 1..1341: mol_type = other DNA
caggtgcagctgttggagtctggcccaggactggtgaagccttcacagaccgtgtccctcacctgcactgtctctggtgtctccatcagcagaggtgtttactcctggagctggatccgccagcacccagggaagggcctcgaatggattgggttcatcgattacaatgggagaaccgactacaacccgtccctcaagagtcgagttaccatatcacaagacacgtctaagaacgacttctccctgaagctgacgtctgtgactgccgcggacacggccatatattactgtgcgagaggtttgcatgcttttgatatctggggccaagggacaatggtcaccgtctcatcagcttccaccaagggcccctccgtgttccccctggctccctcttccaagagcaccagcggcggcaccgctgctctgggatgtctggtgaaggactacttccctgagcctgtgaccgtgtcctggaattccggcgccctgacctccggcgtgcacacattccctgctgtgctgcagtcctccggcctgtatagcctgtcctccgtggtgacagtgcctagctccagcctgggcacccagacctatatctgcaacgtgaaccacaagcctagcaataccaaggtggacaagaaggtggagcctaagagctgcgacaagacccacacctgtcctccatgtcctgctccagaactgctcggcggaccttccgtgttcctgtttcctccaaagcctaaggacaccctgatgatcagcagaacccctgaagtgacctgcgtggtggtggatgtgtcccacgaggatcccgaagtgaagttcaattggtacgtggacggcgtggaagtgcacaacgccaagaccaagcctagagaggaacagtacaacagcacctacagagtggtgtccgtgctgaccgtgctgcaccaggattggctgaacggcaaagagtacaagtgcaaggtgtccaacaaggccctgcctgctcctatcgagaaaaccatcagcaaggccaagggccagcctagggaaccccaggtttacacactgcctccaagcagggacgagctgaccaagaatcaggtgtccctgacctgcctggtcaagggcttctacccttccgatatcgccgtggaatgggagagcaatggccagcctgagaacaactacaagacaacccctcctgtgctggacagcgacggctcattcttcctgtacagcaagctgacagtggacaagagcagatggcagcagggcaacgtgttcagctgcagcgtgatgcacgaggccctgcacaaccactacacccagaagtccctgagcctgtctcctggcaaa

SEQ ID NO: 26 - DNA, 1350 bp, synthetic construct
  source 1..1350: mol_type = other DNA
cggctgcagctgcaggagtcgggcccacgactggtgaagccttcggagaccctgtccctcacctgcagcgtctctggtggctccatcagcagtaggaatcactactgggcctggatccgccagcccccagggaagggcctggagtggattgggtacatctattacagtgggagcacctactacaacccgtccctcaagagtcgagttaccatatcagtagacacgtctaagaaccagttctccctgaagctgagctctgtgactgccgcggacacggccgtgtattactgtgcgagagtagggctgctgctccgggactttgactactggggccagggaaccctggtcaccgtctcatcagcttccaccaagggcccctccgtgttccccctggctccctcttccaagagcaccagcggcggcaccgctgctctgggatgtctggtgaaggactacttccctgagcctgtgaccgtgtcctggaattccggcgccctgacctccggcgtgcacacattccctgctgtgctgcagtcctccggcctgtatagcctgtcctccgtggtgacagtgcctagctccagcctgggcacccagacctatatctgcaacgtgaaccacaagcctagcaataccaaggtggacaagaaggtggagcctaagagctgcgacaagacccacacctgtcctccatgtcctgctccagaactgctcggcggaccttccgtgttcctgtttcctccaaagcctaaggacaccctgatgatcagcagaacccctgaagtgacctgcgtggtggtggatgtgtcccacgaggatcccgaagtgaagttcaattggtacgtggacggcgtggaagtgcacaacgccaagaccaagcctagagaggaacagtacaacagcacctacagagtggtgtccgtgctgaccgtgctgcaccaggattggctgaacggcaaagagtacaagtgcaaggtgtccaacaaggccctgcctgctcctatcgagaaaaccatcagcaaggccaagggccagcctagggaaccccaggtttacacactgcctccaagcagggacgagctgaccaagaatcaggtgtccctgacctgcctggtcaagggcttctacccttccgatatcgccgtggaatgggagagcaatggccagcctgagaacaactacaagacaacccctcctgtgctggacagcgacggctcattcttcctgtacagcaagctgacagtggacaagagcagatggcagcagggcaacgtgttcagctgcagcgtgatgcacgaggccctgcacaaccactacacccagaagtccctgagcctgtctcctggcaaa

SEQ ID NO: 27 - DNA, 1356 bp, synthetic construct
  source 1..1356: mol_type = other DNA
gaggtgcagctggtggagtctgggggaggcgtggtccagcctgggaggtccctgagactctcctgtgcagcctctggattcaccttcagtagctatgctatgcactgggtccgccaggctccaggcaaggggctggagtgggtggcagttatatcatatgatggaagtaataaatactacgcagactccgtgaagggccgattcaccatctccagagacaattccaagaacacgctgtatctgcaaatgaacagcctgagagctgaggacacggctgtgtattactgtgcgagggattgtagtggtggtagctgctatgatgcttttgatatctggggccaagggacaatggtcaccgtctcatcagcttccaccaagggcccctccgtgttccccctggctccctcttccaagagcaccagcggcggcaccgctgctctgggatgtctggtgaaggactacttccctgagcctgtgaccgtgtcctggaattccggcgccctgacctccggcgtgcacacattccctgctgtgctgcagtcctccggcctgtatagcctgtcctccgtggtgacagtgcctagctccagcctgggcacccagacctatatctgcaacgtgaaccacaagcctagcaataccaaggtggacaagaaggtggagcctaagagctgcgacaagacccacacctgtcctccatgtcctgctccagaactgctcggcggaccttccgtgttcctgtttcctccaaagcctaaggacaccctgatgatcagcagaacccctgaagtgacctgcgtggtggtggatgtgtcccacgaggatcccgaagtgaagttcaattggtacgtggacggcgtggaagtgcacaacgccaagaccaagcctagagaggaacagtacaacagcacctacagagtggtgtccgtgctgaccgtgctgcaccaggattggctgaacggcaaagagtacaagtgcaaggtgtccaacaaggccctgcctgctcctatcgagaaaaccatcagcaaggccaagggccagcctagggaaccccaggtttacacactgcctccaagcagggacgagctgaccaagaatcaggtgtccctgacctgcctggtcaagggcttctacccttccgatatcgccgtggaatgggagagcaatggccagcctgagaacaactacaagacaacccctcctgtgctggacagcgacggctcattcttcctgtacagcaagctgacagtggacaagagcagatggcagcagggcaacgtgttcagctgcagcgtgatgcacgaggccctgcacaaccactacacccagaagtccctgagcctgtctcctggcaaa

SEQ ID NO: 28 - DNA, 1353 bp, synthetic construct
  source 1..1353: mol_type = other DNA
caggtgcagctacaggagtcgggcccaggactggtgaagccttcacagaccctgtccctcacctgcactgtctctggtggctccatcagcagtggtggttactactggagctggatccgccagcacccagggaagggcctggagtggattgggtacatctattacagtgggagcacctactacaacccgtccctcaagagtcgagttaccatatcagtagacacgtctaagaaccagttctccctgaagctgagctctgtgactgccgcggacacggccgtgtattactgtgcgagagttggagtagcccttcactacggtatggacgtctggggccaagggaccacggtcaccgtctcatcagcttccaccaagggcccctccgtgttccccctggctccctcttccaagagcaccagcggcggcaccgctgctctgggatgtctggtgaaggactacttccctgagcctgtgaccgtgtcctggaattccggcgccctgacctccggcgtgcacacattccctgctgtgctgcagtcctccggcctgtatagcctgtcctccgtggtgacagtgcctagctccagcctgggcacccagacctatatctgcaacgtgaaccacaagcctagcaataccaaggtggacaagaaggtggagcctaagagctgcgacaagacccacacctgtcctccatgtcctgctccagaactgctcggcggaccttccgtgttcctgtttcctccaaagcctaaggacaccctgatgatcagcagaacccctgaagtgacctgcgtggtggtggatgtgtcccacgaggatcccgaagtgaagttcaattggtacgtggacggcgtggaagtgcacaacgccaagaccaagcctagagaggaacagtacaacagcacctacagagtggtgtccgtgctgaccgtgctgcaccaggattggctgaacggcaaagagtacaagtgcaaggtgtccaacaaggccctgcctgctcctatcgagaaaaccatcagcaaggccaagggccagcctagggaaccccaggtttacacactgcctccaagcagggacgagctgaccaagaatcaggtgtccctgacctgcctggtcaagggcttctacccttccgatatcgccgtggaatgggagagcaatggccagcctgagaacaactacaagacaacccctcctgtgctggacagcgacggctcattcttcctgtacagcaagctgacagtggacaagagcagatggcagcagggcaacgtgttcagctgcagcgtgatgcacgaggccctgcacaaccactacacccagaagtccctgagcctgtctcctggcaaa

SEQ ID NO: 29 - DNA, 1341 bp, synthetic construct
  source 1..1341: mol_type = other DNA
gaggtgcagctggtggagtctgggggagtcgtggtacagcctggggggtccctgagactctcctgtgcagcctctggattcacctttgatgattataccatgcactgggtccgtcaagctccggggaagggtctggagtgggtctctcttattagttgggatggtggtagcacatactatgcagactctgtgaagggccgattcaccatctccagagacaacgccaagaacacgctgtatctgcaaatgaacagtctgagagccgaggacacggctgtgtattactgtgcaagagatacggggtacgctatggatgtctggggccaagggacaatggtcaccgtctcatcagcttccaccaagggcccctccgtgttccccctggctccctcttccaagagcaccagcggcggcaccgctgctctgggatgtctggtgaaggactacttccctgagcctgtgaccgtgtcctggaattccggcgccctgacctccggcgtgcacacattccctgctgtgctgcagtcctccggcctgtatagcctgtcctccgtggtgacagtgcctagctccagcctgggcacccagacctatatctgcaacgtgaaccacaagcctagcaataccaaggtggacaagaaggtggagcctaagagctgcgacaagacccacacctgtcctccatgtcctgctccagaactgctcggcggaccttccgtgttcctgtttcctccaaagcctaaggacaccctgatgatcagcagaacccctgaagtgacctgcgtggtggtggatgtgtcccacgaggatcccgaagtgaagttcaattggtacgtggacggcgtggaagtgcacaacgccaagaccaagcctagagaggaacagtacaacagcacctacagagtggtgtccgtgctgaccgtgctgcaccaggattggctgaacggcaaagagtacaagtgcaaggtgtccaacaaggccctgcctgctcctatcgagaaaaccatcagcaaggccaagggccagcctagggaaccccaggtttacacactgcctccaagcagggacgagctgaccaagaatcaggtgtccctgacctgcctggtcaagggcttctacccttccgatatcgccgtggaatgggagagcaatggccagcctgagaacaactacaagacaacccctcctgtgctggacagcgacggctcattcttcctgtacagcaagctgacagtggacaagagcagatggcagcagggcaacgtgttcagctgcagcgtgatgcacgaggccctgcacaaccactacacccagaagtccctgagcctgtctcctggcaaa

SEQ ID NO: 30 - DNA, 1350 bp, synthetic construct
  source 1..1350: mol_type = other DNA
caggtccagctggtgcagtctggggctgaggtgaagaagcctgggtcctcggtgaaggtctcctgcaaggcttctggaggcaccttcagcagctatgctatcagctgggtgcgacaggcccctggacaagggcttgagtggatgggaaggatcatccctatccttggtatagcaaactacgcacagaagttccagggcagagtcacgattaccgcggacaaatccacgagcacagcctacatggagctgagcagcctgagatctgaggacacggccgtgtattactgtgcgagagcggagggcagcagctggtactactttgactactggggccagggaaccctggtcaccgtctcatcagcttccaccaagggcccctccgtgttccccctggctccctcttccaagagcaccagcggcggcaccgctgctctgggatgtctggtgaaggactacttccctgagcctgtgaccgtgtcctggaattccggcgccctgacctccggcgtgcacacattccctgctgtgctgcagtcctccggcctgtatagcctgtcctccgtggtgacagtgcctagctccagcctgggcacccagacctatatctgcaacgtgaaccacaagcctagcaataccaaggtggacaagaaggtggagcctaagagctgcgacaagacccacacctgtcctccatgtcctgctccagaactgctcggcggaccttccgtgttcctgtttcctccaaagcctaaggacaccctgatgatcagcagaacccctgaagtgacctgcgtggtggtggatgtgtcccacgaggatcccgaagtgaagttcaattggtacgtggacggcgtggaagtgcacaacgccaagaccaagcctagagaggaacagtacaacagcacctacagagtggtgtccgtgctgaccgtgctgcaccaggattggctgaacggcaaagagtacaagtgcaaggtgtccaacaaggccctgcctgctcctatcgagaaaaccatcagcaaggccaagggccagcctagggaaccccaggtttacacactgcctccaagcagggacgagctgaccaagaatcaggtgtccctgacctgcctggtcaagggcttctacccttccgatatcgccgtggaatgggagagcaatggccagcctgagaacaactacaagacaacccctcctgtgctggacagcgacggctcattcttcctgtacagcaagctgacagtggacaagagcagatggcagcagggcaacgtgttcagctgcagcgtgatgcacgaggccctgcacaaccactacacccagaagtccctgagcctgtctcctggcaaa

SEQ ID NO: 31 - DNA, 1350 bp, synthetic construct
  source 1..1350: mol_type = other DNA
cagctgcagctgcaggagtcgggcccaggactggtgaagccttcggggaccctgtccctcacctgcgctgtctctggtggctccatcagcagtagtaactggtggagttgggtccgccagcccccagggaaggggctggagtggattggggaaatctatcatagtgggagcaccaactacaacccgtccctcaagagtcgagtcaccatatcagtagacaagtccaagaaccagttctccctgaagctgagctctgtgaccgccgcggacacggccgtgtattactgtgcgagagcccactcccgatattactatggccttgactactggggccagggaaccctggtcaccgtctcatcagcttccaccaagggcccctccgtgttccccctggctccctcttccaagagcaccagcggcggcaccgctgctctgggatgtctggtgaaggactacttccctgagcctgtgaccgtgtcctggaattccggcgccctgacctccggcgtgcacacattccctgctgtgctgcagtcctccggcctgtatagcctgtcctccgtggtgacagtgcctagctccagcctgggcacccagacctatatctgcaacgtgaaccacaagcctagcaataccaaggtggacaagaaggtggagcctaagagctgcgacaagacccacacctgtcctccatgtcctgctccagaactgctcggcggaccttccgtgttcctgtttcctccaaagcctaaggacaccctgatgatcagcagaacccctgaagtgacctgcgtggtggtggatgtgtcccacgaggatcccgaagtgaagttcaattggtacgtggacggcgtggaagtgcacaacgccaagaccaagcctagagaggaacagtacaacagcacctacagagtggtgtccgtgctgaccgtgctgcaccaggattggctgaacggcaaagagtacaagtgcaaggtgtccaacaaggccctgcctgctcctatcgagaaaaccatcagcaaggccaagggccagcctagggaaccccaggtttacacactgcctccaagcagggacgagctgaccaagaatcaggtgtccctgacctgcctggtcaagggcttctacccttccgatatcgccgtggaatgggagagcaatggccagcctgagaacaactacaagacaacccctcctgtgctggacagcgacggctcattcttcctgtacagcaagctgacagtggacaagagcagatggcagcagggcaacgtgttcagctgcagcgtgatgcacgaggccctgcacaaccactacacccagaagtccctgagcctgtctcctggcaaa

SEQ ID NO: 32 - DNA, 1350 bp, synthetic construct
  source 1..1350: mol_type = other DNA
caggtgcagctacaacagtggggggcagagcttgtgaagccaggggcctcagtcaagttgtcctgcacagcttctggcttcaacattaaagacacctatatgcactgggtgaagcagaggcctgaacagggcctggagtggattggaaggattgatcctgcgaatggtaatactaaatatgacccgaagttccagggcaaggccactataacagcagacacatcctccaacacagcctacctgcagctcagcagcctgacatctgaggacactgccgtctattactgtgctagatcctactataggtacgacgggtacttcgatgtctggggcgcagggacaatggtcaccgtctcatcagcttccaccaagggcccctccgtgttccccctggctccctcttccaagagcaccagcggcggcaccgctgctctgggatgtctggtgaaggactacttccctgagcctgtgaccgtgtcctggaattccggcgccctgacctccggcgtgcacacattccctgctgtgctgcagtcctccggcctgtatagcctgtcctccgtggtgacagtgcctagctccagcctgggcacccagacctatatctgcaacgtgaaccacaagcctagcaataccaaggtggacaagaaggtggagcctaagagctgcgacaagacccacacctgtcctccatgtcctgctccagaactgctcggcggaccttccgtgttcctgtttcctccaaagcctaaggacaccctgatgatcagcagaacccctgaagtgacctgcgtggtggtggatgtgtcccacgaggatcccgaagtgaagttcaattggtacgtggacggcgtggaagtgcacaacgccaagaccaagcctagagaggaacagtacaacagcacctacagagtggtgtccgtgctgaccgtgctgcaccaggattggctgaacggcaaagagtacaagtgcaaggtgtccaacaaggccctgcctgctcctatcgagaaaaccatcagcaaggccaagggccagcctagggaaccccaggtttacacactgcctccaagcagggacgagctgaccaagaatcaggtgtccctgacctgcctggtcaagggcttctacccttccgatatcgccgtggaatgggagagcaatggccagcctgagaacaactacaagacaacccctcctgtgctggacagcgacggctcattcttcctgtacagcaagctgacagtggacaagagcagatggcagcagggcaacgtgttcagctgcagcgtgatgcacgaggccctgcacaaccactacacccagaagtccctgagcctgtctcctggcaaa

SEQ ID NO: 33 - DNA, 1353 bp, synthetic construct
  source 1..1353: mol_type = other DNA
cggctgcagctgcaggagtcgggcccaggactggtgaagccttcggagaccctgtccctcacctgcactgtctctggtggctccatcagcagtagtagttactactggggctggatccgccagcccccagggaaggggctggagtggattgggagtatctattatagtgggagcacctactacaacccgtccctcaagagtcgagtcaccatatccgtagacacgtccaagaaccagttctccctgaagctgagctctgtgaccgccgcagacacggctgtgtattactgtgcgagacggtacagctatggtagagatgcttttgatatctggggccaagggacaatggtcaccgtctcatcagcttccaccaagggcccctccgtgttccccctggctccctcttccaagagcaccagcggcggcaccgctgctctgggatgtctggtgaaggactacttccctgagcctgtgaccgtgtcctggaattccggcgccctgacctccggcgtgcacacattccctgctgtgctgcagtcctccggcctgtatagcctgtcctccgtggtgacagtgcctagctccagcctgggcacccagacctatatctgcaacgtgaaccacaagcctagcaataccaaggtggacaagaaggtggagcctaagagctgcgacaagacccacacctgtcctccatgtcctgctccagaactgctcggcggaccttccgtgttcctgtttcctccaaagcctaaggacaccctgatgatcagcagaacccctgaagtgacctgcgtggtggtggatgtgtcccacgaggatcccgaagtgaagttcaattggtacgtggacggcgtggaagtgcacaacgccaagaccaagcctagagaggaacagtacaacagcacctacagagtggtgtccgtgctgaccgtgctgcaccaggattggctgaacggcaaagagtacaagtgcaaggtgtccaacaaggccctgcctgctcctatcgagaaaaccatcagcaaggccaagggccagcctagggaaccccaggtttacacactgcctccaagcagggacgagctgaccaagaatcaggtgtccctgacctgcctggtcaagggcttctacccttccgatatcgccgtggaatgggagagcaatggccagcctgagaacaactacaagacaacccctcctgtgctggacagcgacggctcattcttcctgtacagcaagctgacagtggacaagagcagatggcagcagggcaacgtgttcagctgcagcgtgatgcacgaggccctgcacaaccactacacccagaagtccctgagcctgtctcctggcaaa

SEQ ID NO: 34 - DNA, 1347 bp, synthetic construct
  source 1..1347: mol_type = other DNA
cagctgcagctgcaggagtcgggcccaggactggtgaagccttcggagaccctgtccctcacctgcactgtctctggtggctccatcagcagtagtagttactactggggctggatccgccagcccccagggaaggggctggagtggattgggagtatctattatagtgggagcacctactacaacccgtccctcaagagtcgagtcaccatatccgtagacacgtccaagaaccagttctccctgaagctgagctctgtgaccgccgcagacacggctgtgtattactgtgcgagactgacgatttttggagtggtgctctactggggccagggaaccctggtcaccgtctcatcagcttccaccaagggcccctccgtgttccccctggctccctcttccaagagcaccagcggcggcaccgctgctctgggatgtctggtgaaggactacttccctgagcctgtgaccgtgtcctggaattccggcgccctgacctccggcgtgcacacattccctgctgtgctgcagtcctccggcctgtatagcctgtcctccgtggtgacagtgcctagctccagcctgggcacccagacctatatctgcaacgtgaaccacaagcctagcaataccaaggtggacaagaaggtggagcctaagagctgcgacaagacccacacctgtcctccatgtcctgctccagaactgctcggcggaccttccgtgttcctgtttcctccaaagcctaaggacaccctgatgatcagcagaacccctgaagtgacctgcgtggtggtggatgtgtcccacgaggatcccgaagtgaagttcaattggtacgtggacggcgtggaagtgcacaacgccaagaccaagcctagagaggaacagtacaacagcacctacagagtggtgtccgtgctgaccgtgctgcaccaggattggctgaacggcaaagagtacaagtgcaaggtgtccaacaaggccctgcctgctcctatcgagaaaaccatcagcaaggccaagggccagcctagggaaccccaggtttacacactgcctccaagcagggacgagctgaccaagaatcaggtgtccctgacctgcctggtcaagggcttctacccttccgatatcgccgtggaatgggagagcaatggccagcctgagaacaactacaagacaacccctcctgtgctggacagcgacggctcattcttcctgtacagcaagctgacagtggacaagagcagatggcagcagggcaacgtgttcagctgcagcgtgatgcacgaggccctgcacaaccactacacccagaagtccctgagcctgtctcctggcaaa

SEQ ID NO: 35 - DNA, 1341 bp, synthetic construct
  source 1..1341: mol_type = other DNA
gaggtgcagctgttggagtctgggggaggcgtggtccagcctgggaggtccctgagactctcctgtgcagcctctggattcaccttcagtagctatgctatgcactgggtccgccaggctccaggcaaggggctggagtgggtggcagttatatcatatgatggaagtaataaatactacgcagactccgtgaagggccgattcaccatctccagagacaattccaagaacacgctgtatctgcaaatgaacagcctgagagctgaggacacggctgtgtattactgtgcgagaggaaagtacaactggttcgacccctggggccagggcaccctggtcaccgtctcatcagcttccaccaagggcccctccgtgttccccctggctccctcttccaagagcaccagcggcggcaccgctgctctgggatgtctggtgaaggactacttccctgagcctgtgaccgtgtcctggaattccggcgccctgacctccggcgtgcacacattccctgctgtgctgcagtcctccggcctgtatagcctgtcctccgtggtgacagtgcctagctccagcctgggcacccagacctatatctgcaacgtgaaccacaagcctagcaataccaaggtggacaagaaggtggagcctaagagctgcgacaagacccacacctgtcctccatgtcctgctccagaactgctcggcggaccttccgtgttcctgtttcctccaaagcctaaggacaccctgatgatcagcagaacccctgaagtgacctgcgtggtggtggatgtgtcccacgaggatcccgaagtgaagttcaattggtacgtggacggcgtggaagtgcacaacgccaagaccaagcctagagaggaacagtacaacagcacctacagagtggtgtccgtgctgaccgtgctgcaccaggattggctgaacggcaaagagtacaagtgcaaggtgtccaacaaggccctgcctgctcctatcgagaaaaccatcagcaaggccaagggccagcctagggaaccccaggtttacacactgcctccaagcagggacgagctgaccaagaatcaggtgtccctgacctgcctggtcaagggcttctacccttccgatatcgccgtggaatgggagagcaatggccagcctgagaacaactacaagacaacccctcctgtgctggacagcgacggctcattcttcctgtacagcaagctgacagtggacaagagcagatggcagcagggcaacgtgttcagctgcagcgtgatgcacgaggccctgcacaaccactacacccagaagtccctgagcctgtctcctggcaaa

SEQ ID NO: 36 - DNA, 1344 bp, synthetic construct
  source 1..1344: mol_type = other DNA
caggtgcagctggtggactctggggggggcttggtacagcctggagggtccctgagactctcctgtgtagcctctggattcgccttcagtaattatgagatgaactgggtccgccaggctccagggaaggggctggagtgggtttcatacattagtagtagtagtagttacacaaactacgcagactctgtgaagggccgattcaccatctccagagacaacgccaagaactcactgtatctgcaaatgaacagcctgagagccgaggacacggccgtgtattactgtgcgagagcccaggttcgggatgcttttgatatctggggccaagggaccacggtcaccgtctcatcagcttccaccaagggcccctccgtgttccccctggctccctcttccaagagcaccagcggcggcaccgctgctctgggatgtctggtgaaggactacttccctgagcctgtgaccgtgtcctggaattccggcgccctgacctccggcgtgcacacattccctgctgtgctgcagtcctccggcctgtatagcctgtcctccgtggtgacagtgcctagctccagcctgggcacccagacctatatctgcaacgtgaaccacaagcctagcaataccaaggtggacaagaaggtggagcctaagagctgcgacaagacccacacctgtcctccatgtcctgctccagaactgctcggcggaccttccgtgttcctgtttcctccaaagcctaaggacaccctgatgatcagcagaacccctgaagtgacctgcgtggtggtggatgtgtcccacgaggatcccgaagtgaagttcaattggtacgtggacggcgtggaagtgcacaacgccaagaccaagcctagagaggaacagtacaacagcacctacagagtggtgtccgtgctgaccgtgctgcaccaggattggctgaacggcaaagagtacaagtgcaaggtgtccaacaaggccctgcctgctcctatcgagaaaaccatcagcaaggccaagggccagcctagggaaccccaggtttacacactgcctccaagcagggacgagctgaccaagaatcaggtgtccctgacctgcctggtcaagggcttctacccttccgatatcgccgtggaatgggagagcaatggccagcctgagaacaactacaagacaacccctcctgtgctggacagcgacggctcattcttcctgtacagcaagctgacagtggacaagagcagatggcagcagggcaacgtgttcagctgcagcgtgatgcacgaggccctgcacaaccactacacccagaagtccctgagcctgtctcctggcaaa

SEQ ID NO: 37 - protein, 107 aa, synthetic construct
DIQLTQSPSSLSASVGDRVTITCRASQSIISYLNWYQQKPGKAPKLLIYAASSLQSGVPSRFSGSGSGTDFTLTISSLQPEDFATYYCQQSYSTPDTFGQGTKLEIK

SEQ ID NO: 38 - protein, 11 aa, synthetic construct
RASQSIISYLN

SEQ ID NO: 39 - protein, 7 aa, synthetic construct
AASSLQS

SEQ ID NO: 40 - protein, 9 aa, synthetic construct
QQSYSTPDT

SEQ ID NO: 41 - protein, 107 aa, synthetic construct
EIVLTQSPATLSLSPGERATLSCRASQSVSSNLGWYQQKPGQAPSLLIYGASNRATGIPARFSGSGSGTDFTLTISSLEPEDFAVYYCQQRDTWPLTFGGGTKVEIK

SEQ ID NO: 42 - protein, 11 aa, synthetic construct
RASQSVSSNLG

SEQ ID NO: 43 - protein, 7 aa, synthetic construct
GASNRAT

SEQ ID NO: 44 - protein, 9 aa, synthetic construct
QQRDTWPLT

SEQ ID NO: 45 - protein, 107 aa, synthetic construct
EIVLTQSPATLPLSPGERATLSCRASQSVGFYLAWYQQKPGQPPRLLFYDASKRATGIPARFSASGSGTDFTLTISGLEPEDFAVYYCQHRISWPLTFGQGTKVEVK

SEQ ID NO: 46 - protein, 11 aa, synthetic construct
RASQSVGFYLA

SEQ ID NO: 47 - protein, 7 aa, synthetic construct
DASKRAT

SEQ ID NO: 48 - protein, 9 aa, synthetic construct
QHRISWPLT

SEQ ID NO: 49 - protein, 107 aa, synthetic construct
EIVLTQSPATLSLSPGERATLSCRASQSVSTYLAWYQQKPGQAPRLLIYDTSIRATGIPARFSGSGSGTDFTLTISSLEPEDFAVYYCQQRSNWPLTFGGGTKVEIK

SEQ ID NO: 50 - protein, 11 aa, synthetic construct
RASQSVSTYLA

SEQ ID NO: 51 - protein, 7 aa, synthetic construct
DTSIRAT

SEQ ID NO: 52 - protein, 9 aa, synthetic construct
QQRSNWPLT

SEQ ID NO: 53 - protein, 107 aa, synthetic construct
EIVLTQSPAILSLSPGERATLSCRASQSVSEYLAWYQQKPGQAPRLLIYDISNRATGIPARFSGSGSETDFTLTISSLEPEDFAVYYCQQRRTWPLTFGPGTKVDIK

SEQ ID NO: 54 - protein, 11 aa, synthetic construct
RASQSVSEYLA

SEQ ID NO: 55 - protein, 7 aa, synthetic construct
DISNRAT

SEQ ID NO: 56 - protein, 9 aa, synthetic construct
QQRRTWPLT

SEQ ID NO: 57 - protein, 107 aa, synthetic construct
NIQLTQSPPFLSASVGDRVTITCRASQDISSFLAWYQQKPGKAPNLLIHAATTLQSGVPSRFSGSGSGTEFTLTISSLRPEDFATYYCQQLHTYPITFGQGTRLEIK

SEQ ID NO: 58 - protein, 11 aa, synthetic construct
RASQDISSFLA

SEQ ID NO: 59 - protein, 7 aa, synthetic construct
AATTLQS

SEQ ID NO: 60 - protein, 9 aa, synthetic construct
QQLHTYPIT

SEQ ID NO: 61 - protein, 106 aa, synthetic construct
NIQMTQSPPSLSASVGDRVAITCRASQDISNSLAWYQQKSGQPPKLLLYDVSKLERGVPSRFSGSGSRTDYTLTISSLQPEDFATYYCQQYSSDPTFGQGSKLEFK

SEQ ID NO: 62 - protein, 11 aa, synthetic construct
RASQDISNSLA

SEQ ID NO: 63 - protein, 7 aa, synthetic construct
DVSKLER

SEQ ID NO: 64 - protein, 8 aa, synthetic construct
QQYSSDPT

SEQ ID NO: 65 - protein, 107 aa, synthetic construct
DIQMIQSPSSVSASVGDRVTITCRASQGISNSLAWYQHKPGTTPKLLIYAASSLQGGVPSRFSGSSSETDFTLTISSLQPEDFATYYCQQANSFPITFGQGTRLDIK

SEQ ID NO: 66 - protein, 11 aa, synthetic construct
RASQGISNSLA

SEQ ID NO: 67 - protein, 7 aa, synthetic construct
AASSLQG

SEQ ID NO: 68 - protein, 9 aa, synthetic construct
QQANSFPIT

SEQ ID NO: 69 - protein, 108 aa, synthetic construct
EIVLTQSPATLSLSPGERATLSCRASQSVSSYLAWYQQKPGQAPRLLIYDASNRATGIPARFSGSGSGTDFTLTISSLEPEDFAVYYCQQRTNWLMYTFGQGTKLEIK

SEQ ID NO: 70 - protein, 11 aa, synthetic construct
RASQSVSSYLA

SEQ ID NO: 71 - protein, 7 aa, synthetic construct
DASNRAT

SEQ ID NO: 72 - protein, 10 aa, synthetic construct
QQRTNWLMYT

SEQ ID NO: 73 - protein, 107 aa, synthetic construct
EIVLTQSPATLSLSPGERATLSCRASQSVSSYLAWYQQKPGQAPRLLIYDASNRATGIPARFSGSGSGTDFTLTISSLEPEDFAVYYCQQRSNWPLTFGGGTKVEIK

SEQ ID NO: 74 - protein, 11 aa, synthetic construct
RASQSVSSYLA

SEQ ID NO: 75 - protein, 7 aa, synthetic construct
DASNRAT

SEQ ID NO: 76 - protein, 9 aa, synthetic construct
QQRSNWPLT

SEQ ID NO: 77 - protein, 106 aa, synthetic construct
NIQMTQSPSSLSASVGDRVTITCRASQSISSYLNWYQQKPGKAPKLLIYAASSLQSGVPSRFSGSGSGTDFTLTISSLQPEDFASYYCQQSYSSWAFGQGTKVEIK

SEQ ID NO: 78 - protein, 11 aa, synthetic construct
RASQSISSYLN

SEQ ID NO: 79 - protein, 7 aa, synthetic construct
AASSLQS

SEQ ID NO: 80 - protein, 8 aa, synthetic construct
QQSYSSWA

SEQ ID NO: 81 - protein, 107 aa, synthetic construct
NIQLTQSPSSVSASVGDRVTITCRASQGFSRWLAWYQQKPGKAPKLLIYGASSLQSGVPSRFSGSGSGTDFTLTISSLQPEDFATYYCQQANSFPLTFGGGTKLEIK

SEQ ID NO: 82 - protein, 11 aa, synthetic construct
RASQGFSRWLA

SEQ ID NO: 83 - protein, 7 aa, synthetic construct
GASSLQS

SEQ ID NO: 84 - protein, 9 aa, synthetic construct
QQANSFPLT

SEQ ID NO: 85 - protein, 107 aa, synthetic construct
NIQLTQSPSSLSASVGDRVTITCRASQSISSYLNWYQQKPGKAPKLLIYAASSLQSGVPSRFSGSGSGTDFTLTISSLQPEDFATYYCQQSYSTPDTFGPGTKVDIK

SEQ ID NO: 86 - protein, 11 aa, synthetic construct
RASQSISSYLN

SEQ ID NO: 87 - protein, 7 aa, synthetic construct
AASSLQS

SEQ ID NO: 88 - protein, 9 aa, synthetic construct
QQSYSTPDT

SEQ ID NO: 89 - protein, 110 aa, synthetic construct
QSALTQPASVSGSPGQSITISCTGTSSDVGGYNYVSWYQQHPGKAPKLMIYDVSNRPSGVSNRFSGSKSGNTASLTISGLQAEDEADYYCSSFTTITTRVFGGGTKLTVL

SEQ ID NO: 90 - protein, 14 aa, synthetic construct
TGTSSDVGGYNYVS

SEQ ID NO: 91 - protein, 7 aa, synthetic construct
DVSNRPS

SEQ ID NO: 92 - protein, 10 aa, synthetic construct
SSFTTITTRV

SEQ ID NO: 93 - protein, 110 aa, synthetic construct
QSALTQPASVSGSPGQSITISCSGTSSDIGRYNYVSWYQQHPGKAPKLLIFDVSNRPSGVSNRFSGSKSGNTASLTISGLQAEDEADYYCSSYTSTVPYVFGTGTRVAVQ

SEQ ID NO: 94 - protein, 14 aa, synthetic construct
SGTSSDIGRYNYVS

SEQ ID NO: 95 - protein, 7 aa, synthetic construct
DVSNRPS

SEQ ID NO: 96 - protein, 10 aa, synthetic construct
SSYTSTVPYV

SEQ ID NO: 97 - protein, 109 aa, synthetic construct
EIVLTQSPATLSLSPGERATLSCQASQTFSDYLAWYQQKPGQAPRLLIYDASTRATGIPARFSGSGSGTDFTLTISSLEPEDFAVYYCQQRSHWPPGYTFGQGTRVEIK

SEQ ID NO: 98 - protein, 11 aa, synthetic construct
QASQTFSDYLA

SEQ ID NO: 99 - protein, 7 aa, synthetic construct
DASTRAT

SEQ ID NO: 100 - protein, 11 aa, synthetic construct
QQRSHWPPGYT

SEQ ID NO: 101 - protein, 107 aa, synthetic construct
EIVLTQSPATLSLSPGERATLSCRASQSVYSSLAWYQQKPGQAPKLLIYDASNRATGVPARFSGSGSGTDFTLTISSLEPEDFALYYCQHRQHWPLTFGGGTKVEIK

SEQ ID NO: 102 - protein, 11 aa, synthetic construct
RASQSVYSSLA

SEQ ID NO: 103 - protein, 7 aa, synthetic construct
DASNRAT

SEQ ID NO: 104 - protein, 9 aa, synthetic construct
QHRQHWPLT

SEQ ID NO: 105 - protein, 107 aa, synthetic construct
EIVMTQSPVTLSVSPGDSATLSCRASQSVDKNLAWYQQKTGQAPRLLIYGAATRATGIPARFSGSGSGTEFTLTISSLRSEDFAVYYCQQYRNWPWTFGLGTKVEIK

SEQ ID NO: 106 - protein, 11 aa, synthetic construct
RASQSVDKNLA

SEQ ID NO: 107 - protein, 7 aa, synthetic construct
GAATRAT

SEQ ID NO: 108 - protein, 9 aa, synthetic construct
QQYRNWPWT

SEQ ID NO: 109 - protein, 107 aa, synthetic construct [sequence omitted]

SEQ ID NO: 110 - protein, 106 aa, synthetic construct
GQPKAAPSVTLFPPSSEELQANKATLVCLISDFYPGAVTVAWKADSSPVKAGVETTTPSKQSNNKYAASSYLSLTPEQWKSHRSYSCQVTHEGSTVEKTVAPTECS

SEQ ID NO: 111 - protein, 122 aa, synthetic construct
QVQLVQSGAEVKKPGASVKVSCKASGYTFTSYYMHWVRQAPGQGLEWMGIINPSGGSTSYAQKFQGRVTMTRDTSTSTVYMELSSLRSEDTAVYYCARDISGSYQTDAFDIWGQGTMVTVSS

SEQ ID NO: 112 - protein, 10 aa, synthetic construct
GYTFTSYYMH

SEQ ID NO: 113 - protein, 10 aa, synthetic construct
IINPSGGSTS

SEQ ID NO: 114 - protein, 13 aa, synthetic construct
DISGSYQTDAFDI

SEQ ID NO: 115 - protein, 121 aa, synthetic construct
QVQLQDSGPGLVKPSQTLSLTCTVSGGSISSGGYYWSWIRQHPGKGLEWIGYIYYSGSTYYNPSLKSRVTISVDTSKNQFSLKLSSVTAADTAVYYCARVPVPLVGAFDIWGQGTMVTVSS

SEQ ID NO: 116 - protein, 12 aa, synthetic construct
GGSISSGGYYWS

SEQ ID NO: 117 - protein, 9 aa, synthetic construct
YIYYSGSTY

SEQ ID NO: 118 - protein, 11 aa, synthetic construct
VPVPLVGAFDI

SEQ ID NO: 119 - protein, 119 aa, synthetic construct
RLQLQESGPGLVKPSQTLSLTCTVSGGSISSGGYYWSWIRQHPGKGLEWIGYIYYSGSTYYNPSLKSRVTISVDTSKNQFSLKLSSVTAADTAVYYCARATIYGYFDYWGQGTLVTVSS

SEQ ID NO: 120 - protein, 12 aa, synthetic construct
GGSISSGGYYWS

SEQ ID NO: 121 - protein, 9 aa, synthetic construct
YIYYSGSTY

SEQ ID NO: 122 - protein, 9 aa, synthetic construct
ATIYGYFDY

SEQ ID NO: 123 - protein, 120 aa, synthetic construct
QVQLQESGPGLVKPSQTLSLTCTVSGGSISSGGYYWSWIRQHPGKGLEWIGYIYYSGSTYYNPSLKSRVTISVDTSKNQFSLKLSSVTAADTAVYYCARVRLLGGGFDIWGQGTTVTVSS

SEQ ID NO: 124 - protein, 12 aa, synthetic construct
GGSISSGGYYWS

SEQ ID NO: 125 - protein, 9 aa, synthetic construct
YIYYSGSTY

SEQ ID NO: 126 - protein, 10 aa, synthetic construct
VRLLGGGFDI

SEQ ID NO: 127 - protein, 124 aa, synthetic construct
EVQLVESGGGVVQPGRSLRLSCAASGFTFSSYAMHWVRQAPGKGLEWVAVISYDGSNKYYVDSVKGRFTISRDNSKNTLYLQMNSLRAEDTAVYYCARDRITYLDYYYYGMDVWGQGTTVTVSS

SEQ ID NO: 128 - protein, 10 aa, synthetic construct
GFTFSSYAMH

SEQ ID NO: 129 - protein, 10 aa, synthetic construct
VISYDGSNKY

SEQ ID NO: 130 - protein, 15 aa, synthetic construct
DRITYLDYYYYGMDV

SEQ ID NO: 131 - protein, 120 aa, synthetic construct
QVQLQQSGPGLVKPSQTLSLTCAISGDSVSSDSAAWNWIRQSPSRGLEWLGRTYYRSKWYNDYAVSVKSRITINPDTSKNQFSLQLNSVTSDDTAVYYCARGSWAAPWLWGQGTLVTVSS

SEQ ID NO: 132 - protein, 12 aa, synthetic construct
GDSVSSDSAAWN

SEQ ID NO: 133 - protein, 11 aa, synthetic construct
RTYYRSKWYND

SEQ ID NO: 134 - protein, 8 aa, synthetic construct
GSWAAPWL

SEQ ID NO: 135 - protein, 117 aa, synthetic construct
QVQLLESGPGLVKPSQTVSLTCTVSGVSISRGVYSWSWIRQHPGKGLEWIGFIDYNGRTDYNPSLKSRVTISQDTSKNDFSLKLTSVTAADTAIYYCARGLHAFDIWGQGTMVTVSS

SEQ ID NO: 136 - protein, 12 aa, synthetic construct
GVSISRGVYSWS

SEQ ID NO: 137 - protein, 9 aa, synthetic construct
FIDYNGRTD

SEQ ID NO: 138 - protein, 7 aa, synthetic construct
GLHAFDI

SEQ ID NO: 139 - protein, 120 aa, synthetic construct
RLQLQESGPRLVKPSETLSLTCSVSGGSISSRNHYWAWIRQPPGKGLEWIGYIYYSGSTYYNPSLKSRVTISVDTSKNQFSLKLSSVTAADTAVYYCARVGLLLRDFDYWGQGTLVTVSS

SEQ ID NO: 140 - protein, 12 aa, synthetic construct
GGSISSRNHYWA

SEQ ID NO: 141 - protein, 9 aa, synthetic construct
YIYYSGSTY

SEQ ID NO: 142 - protein, 10 aa, synthetic construct
VGLLLRDFDY

SEQ ID NO: 143 - protein, 122 aa, synthetic construct
EVQLVESGGGVVQPGRSLRLSCAASGFTFSSYAMHWVRQAPGKGLEWVAVISYDGSNKYYADSVKGRFTISRDNSKNTLYLQMNSLRAEDTAVYYCARDCSGGSCYDAFDIWGQGTMVTVSS

SEQ ID NO: 144 - protein, 10 aa, synthetic construct
GFTFSSYAMH

SEQ ID NO: 145 - protein, 10 aa, synthetic construct
VISYDGSNKY

SEQ ID NO: 146 - protein, 13 aa, synthetic construct
DCSGGSCYDAFDI

SEQ ID NO: 147 - protein, 121 aa, synthetic construct
QVQLQESGPGLVKPSQTLSLTCTVSGGSISSGGYYWSWIRQHPGKGLEWIGYIYYSGSTYYNPSLKSRVTISVDTSKNQFSLKLSSVTAADTAVYYCARVGVALHYGMDVWGQGTTVTVSS

SEQ ID NO: 148 - protein, 12 aa, synthetic construct
GGSISSGGYYWS

SEQ ID NO: 149 - protein, 9 aa, synthetic construct
YIYYSGSTY

SEQ ID NO: 150 - protein, 11 aa, synthetic construct
VGVALHYGMDV

SEQ ID NO: 151 - protein, 117 aa, synthetic construct
EVQLVESGGVVVQPGGSLRLSCAASGFTFDDYTMHWVRQAPGKGLEWVSLISWDGGSTYYADSVKGRFTISRDNAKNTLYLQMNSLRAEDTAVYYCARDTGYAMDVWGQGTMVTVSS

SEQ ID NO: 152 - protein, 10 aa, synthetic construct
GFTFDDYTMH

SEQ ID NO: 153 - protein, 10 aa, synthetic construct
LISWDGGSTY

SEQ ID NO: 154 - protein, 8 aa, synthetic construct
DTGYAMDV

SEQ ID NO: 155 - protein, 120 aa, synthetic construct
QVQLVQSGAEVKKPGSSVKVSCKASGGTFSSYAISWVRQAPGQGLEWMGRIIPILGIANYAQKFQGRVTITADKSTSTAYMELSSLRSEDTAVYYCARAEGSSWYYFDYWGQGTLVTVSS

SEQ ID NO: 156 - protein, 10 aa, synthetic construct
GGTFSSYAIS

SEQ ID NO: 157 - protein, 10 aa, synthetic construct
RIIPILGIAN

SEQ ID NO: 158 - protein, 11 aa, synthetic construct
AEGSSWYYFDY

SEQ ID NO: 159 - protein, 120 aa, synthetic construct
QLQLQESGPGLVKPSGTLSLTCAVSGGSISSSNWWSWVRQPPGKGLEWIGEIYHSGSTNYNPSLKSRVTISVDKSKNQFSLKLSSVTAADTAVYYCARAHSRYYYGLDYWGQGTLVTVSS

SEQ ID NO: 160 - protein, 11 aa, synthetic construct
GGSISSSNWWS

SEQ ID NO: 161 - protein, 9 aa, synthetic construct
EIYHSGSTN

SEQ ID NO: 162 - protein, 11 aa, synthetic construct
AHSRYYYGLDY

SEQ ID NO: 163 - protein, 120 aa, synthetic construct
QVQLQQWGAELVKPGASVKLSCTASGFNIKDTYMHWVKQRPEQGLEWIGRIDPANGNTKYDPKFQGKATITADTSSNTAYLQLSSLTSEDTAVYYCARSYYRYDGYFDVWGAGTMVTVSS

SEQ ID NO: 164 - protein, 10 aa, synthetic construct
GFNIKDTYMH

SEQ ID NO: 165 - protein, 10 aa, synthetic construct
RIDPANGNTK

SEQ ID NO: 166 - protein, 11 aa, synthetic construct
SYYRYDGYFDV

SEQ ID NO: 167 - protein, 121 aa, synthetic construct
RLQLQESGPGLVKPSETLSLTCTVSGGSISSSSYYWGWIRQPPGKGLEWIGSIYYSGSTYYNPSLKSRVTISVDTSKNQFSLKLSSVTAADTAVYYCARRYSYGRDAFDIWGQGTMVTVSS

SEQ ID NO: 168 - protein, 12 aa, synthetic construct
GGSISSSSYYWG

SEQ ID NO: 169 - protein, 9 aa, synthetic construct
SIYYSGSTY

SEQ ID NO: 170 - protein, 11 aa, synthetic construct
RYSYGRDAFDI

SEQ ID NO: 171 - protein, 119 aa, synthetic construct
QLQLQESGPGLVKPSETLSLTCTVSGGSISSSSYYWGWIRQPPGKGLEWIGSIYYSGSTYYNPSLKSRVTISVDTSKNQFSLKLSSVTAADTAVYYCARLTIFGVVLYWGQGTLVTVSS

SEQ ID NO: 172 - protein, 12 aa, synthetic construct
GGSISSSSYYWG

SEQ ID NO: 173 - protein, 9 aa, synthetic construct
SIYYSGSTY

SEQ ID NO: 174 - protein, 9 aa, synthetic construct
LTIFGVVLY

SEQ ID NO: 175 - protein, 117 aa, synthetic construct
EVQLLESGGGVVQPGRSLRLSCAASGFTFSSYAMHWVRQAPGKGLEWVAVISYDGSNKYYADSVKGRFTISRDNSKNTLYLQMNSLRAEDTAVYYCARGKYNWFDPWGQGTLVTVSS

SEQ ID NO: 176 - protein, 10 aa, synthetic construct
GFTFSSYAMH

SEQ ID NO: 177 - protein, 10 aa, synthetic construct
VISYDGSNKY

SEQ ID NO: 178 - protein, 8 aa, synthetic construct
GKYNWFDP

SEQ ID NO: 179 - protein, 118 aa, synthetic construct
QVQLVDSGGGLVQPGGSLRLSCVASGFAFSNYEMNWVRQAPGKGLEWVSYISSSSSYTNYADSVKGRFTISRDNAKNSLYLQMNSLRAEDTAVYYCARAQVRDAFDIWGQGTTVTVSS

SEQ ID NO: 180 - protein, 10 aa, synthetic construct
GFAFSNYEMN

SEQ ID NO: 181 - protein, 10 aa, synthetic construct
YISSSSSYTN

SEQ ID NO: 182 - protein, 9 aa, synthetic construct
AQVRDAFDI

SEQ ID NO: 183 - protein, 330 aa, synthetic construct [sequence omitted]

SEQ ID NO: 184 - protein, 214 aa, synthetic construct
DIQLTQSPSSLSASVGDRVTITCRASQSIISYLNWYQQKPGKAPKLLIYAASSLQSGVPSRFSGSGSGTDFTLTISSLQPEDFATYYCQQSYSTPDTFGQGTKLEIKRTVAAPSVFIFPPSDEQLKSGTASVVCLLNNFYPREAKVQWKVDNALQSGNSQESVTEQDSKDSTYSLSSTLTLSKADYEKHKVYACEVTHQGLSSPVTKSFNRGEC

SEQ ID NO: 185 - protein, 214 aa, synthetic construct
EIVLTQSPATLSLSPGERATLSCRASQSVSSNLGWYQQKPGQAPSLLIYGASNRATGIPARFSGSGSGTDFTLTISSLEPEDFAVYYCQQRDTWPLTFGGGTKVEIKRTVAAPSVFIFPPSDEQLKSGTASVVCLLNNFYPREAKVQWKVDNALQSGNSQESVTEQDSKDSTYSLSSTLTLSKADYEKHKVYACEVTHQGLSSPVTKSFNRGEC

SEQ ID NO: 186 - protein, 214 aa, synthetic construct
EIVLTQSPATLPLSPGERATLSCRASQSVGFYLAWYQQKPGQPPRLLFYDASKRATGIPARFSASGSGTDFTLTISGLEPEDFAVYYCQHRISWPLTFGQGTKVEVKRTVAAPSVFIFPPSDEQLKSGTASVVCLLNNFYPREAKVQWKVDNALQSGNSQESVTEQDSKDSTYSLSSTLTLSKADYEKHKVYACEVTHQGLSSPVTKSFNRGEC

SEQ ID NO: 187 - protein, 214 aa, synthetic construct
EIVLTQSPATLSLSPGERATLSCRASQSVSTYLAWYQQKPGQAPRLLIYDTSIRATGIPARFSGSGSGTDFTLTISSLEPEDFAVYYCQQRSNWPLTFGGGTKVEIKRTVAAPSVFIFPPSDEQLKSGTASVVCLLNNFYPREAKVQWKVDNALQSGNSQESVTEQDSKDSTYSLSSTLTLSKADYEKHKVYACEVTHQGLSSPVTKSFNRGEC

SEQ ID NO: 188 - protein, 214 aa, synthetic construct
EIVLTQSPAILSLSPGERATLSCRASQSVSEYLAWYQQKPGQAPRLLIYDISNRATGIPARFSGSGSETDFTLTISSLEPEDFAVYYCQQRRTWPLTFGPGTKVDIKRTVAAPSVFIFPPSDEQLKSGTASVVCLLNNFYPREAKVQWKVDNALQSGNSQESVTEQDSKDSTYSLSSTLTLSKADYEKHKVYACEVTHQGLSSPVTKSFNRGEC

SEQ ID NO: 189 - protein, 214 aa, synthetic construct
NIQLTQSPPFLSASVGDRVTITCRASQDISSFLAWYQQKPGKAPNLLIHAATTLQSGVPSRFSGSGSGTEFTLTISSLRPEDFATYYCQQLHTYPITFGQGTRLEIKRTVAAPSVFIFPPSDEQLKSGTASVVCLLNNFYPREAKVQWKVDNALQSGNSQESVTEQDSKDSTYSLSSTLTLSKADYEKHKVYACEVTHQGLSSPVTKSFNRGEC

SEQ ID NO: 190 - protein, 213 aa, synthetic construct
NIQMTQSPPSLSASVGDRVAITCRASQDISNSLAWYQQKSGQPPKLLLYDVSKLERGVPSRFSGSGSRTDYTLTISSLQPEDFATYYCQQYSSDPTFGQGSKLEFKRTVAAPSVFIFPPSDEQLKSGTASVVCLLNNFYPREAKVQWKVDNALQSGNSQESVTEQDSKDSTYSLSSTLTLSKADYEKHKVYACEVTHQGLSSPVTKSFNRGEC

SEQ ID NO: 191 - protein, 214 aa, synthetic construct
DIQMIQSPSSVSASVGDRVTITCRASQGISNSLAWYQHKPGTTPKLLIYAASSLQGGVPSRFSGSSSETDFTLTISSLQPEDFATYYCQQANSFPITFGQGTRLDIKRTVAAPSVFIFPPSDEQLKSGTASVVCLLNNFYPREAKVQWKVDNALQSGNSQESVTEQDSKDSTYSLSSTLTLSKADYEKHKVYACEVTHQGLSSPVTKSFNRGEC

SEQ ID NO: 192 - protein, 215 aa, synthetic construct
EIVLTQSPATLSLSPGERATLSCRASQSVSSYLAWYQQKPGQAPRLLIYDASNRATGIPARFSGSGSGTDFTLTISSLEPEDFAVYYCQQRTNWLMYTFGQGTKLEIKRTVAAPSVFIFPPSDEQLKSGTASVVCLLNNFYPREAKVQWKVDNALQSGNSQESVTEQDSKDSTYSLSSTLTLSKADYEKHKVYACEVTHQGLSSPVTKSFNRGEC

SEQ ID NO: 193 - protein, 214 aa, synthetic construct
EIVLTQSPATLSLSPGERATLSCRASQSVSSYLAWYQQKPGQAPRLLIYDASNRATGIPARFSGSGSGTDFTLTISSLEPEDFAVYYCQQRSNWPLTFGGGTKVEIKRTVAAPSVFIFPPSDEQLKSGTASVVCLLNNFYPREAKVQWKVDNALQSGNSQESVTEQDSKDSTYSLSSTLTLSKADYEKHKVYACEVTHQGLSSPVTKSFNRGEC

SEQ ID NO: 194 - protein, 213 aa, synthetic construct
NIQMTQSPSSLSASVGDRVTITCRASQSISSYLNWYQQKPGKAPKLLIYAASSLQSGVPSRFSGSGSGTDFTLTISSLQPEDFASYYCQQSYSSWAFGQGTKVEIKRTVAAPSVFIFPPSDEQLKSGTASVVCLLNNFYPREAKVQWKVDNALQSGNSQESVTEQDSKDSTYSLSSTLTLSKADYEKHKVYACEVTHQGLSSPVTKSFNRGEC

SEQ ID NO: 195 - protein, 214 aa, synthetic construct
NIQLTQSPSSVSASVGDRVTITCRASQGFSRWLAWYQQKPGKAPKLLIYGASSLQSGVPSRFSGSGSGTDFTLTISSLQPEDFATYYCQQANSFPLTFGGGTKLEIKRTVAAPSVFIFPPSDEQLKSGTASVVCLLNNFYPREAKVQWKVDNALQSGNSQESVTEQDSKDSTYSLSSTLTLSKADYEKHKVYACEVTHQGLSSPVTKSFNRGEC

SEQ ID NO: 196 - protein, 214 aa, synthetic construct
NIQLTQSPSSLSASVGDRVTITCRASQSISSYLNWYQQKPGKAPKLLIYAASSLQSGVPSRFSGSGSGTDFTLTISSLQPEDFATYYCQQSYSTPDTFGPGTKVDIKRTVAAPSVFIFPPSDEQLKSGTASVVCLLNNFYPREAKVQWKVDNALQSGNSQESVTEQDSKDSTYSLSSTLTLSKADYEKHKVYACEVTHQGLSSPVTKSFNRGEC

SEQ ID NO: 197 - protein, 216 aa, synthetic construct
QSALTQPASVSGSPGQSITISCTGTSSDVGGYNYVSWYQQHPGKAPKLMIYDVSNRPSGVSNRFSGSKSGNTASLTISGLQAEDEADYYCSSFTTITTRVFGGGTKLTVLGQPKAAPSVTLFPPSSEELQANKATLVCLISDFYPGAVTVAWKADSSPVKAGVETTTPSKQSNNKYAASSYLSLTPEQWKSHRSYSCQVTHEGSTVEKTVAPTECS

SEQ ID NO: 198 - protein, 216 aa, synthetic construct
QSALTQPASVSGSPGQSITISCSGTSSDIGRYNYVSWYQQHPGKAPKLLIFDVSNRPSGVSNRFSGSKSGNTASLTISGLQAEDEADYYCSSYTSTVPYVFGTGTRVAVQGQPKAAPSVTLFPPSSEELQANKATLVCLISDFYPGAVTVAWKADSSPVKAGVETTTPSKQSNNKYAASSYLSLTPEQWKSHRSYSCQVTHEGSTVEKTVAPTECS

SEQ ID NO: 199 - protein, 216 aa, synthetic construct
EIVLTQSPATLSLSPGERATLSCQASQTFSDYLAWYQQKPGQAPRLLIYDASTRATGIPARFSGSGSGTDFTLTISSLEPEDFAVYYCQQRSHWPPGYTFGQGTRVEIKRTVAAPSVFIFPPSDEQLKSGTASVVCLLNNFYPREAKVQWKVDNALQSGNSQESVTEQDSKDSTYSLSSTLTLSKADYEKHKVYACEVTHQGLSSPVTKSFNRGEC

SEQ ID NO: 200 - protein, 214 aa, synthetic construct
EIVLTQSPATLSLSPGERATLSCRASQSVYSSLAWYQQKPGQAPKLLIYDASNRATGVPARFSGSGSGTDFTLTISSLEPEDFALYYCQHRQHWPLTFGGGTKVEIKRTVAAPSVFIFPPSDEQLKSGTASVVCLLNNFYPREAKVQWKVDNALQSGNSQESVTEQDSKDSTYSLSSTLTLSKADYEKHKVYACEVTHQGLSSPVTKSFNRGEC

SEQ ID NO: 201 - protein, 213 aa, synthetic construct
IVMTQSPVTLSVSPGDSATLSCRASQSVDKNLAWYQQKTGQAPRLLIYGAATRATGIPARFSGSGSGTEFTLTISSLRSEDFAVYYCQQYRNWPWTFGLGTKVEIKRTVAAPSVFIFPPSDEQLKSGTASVVCLLNNFYPREAKVQWKVDNALQSGNSQESVTEQDSKDSTYSLSSTLTLSKADYEKHKVYACEVTHQGLSSPVTKSFNRGEC

SEQ ID NO: 202 - protein, 452 aa, synthetic construct
QVQLVQSGAEVKKPGASVKVSCKASGYTFTSYYMHWVRQAPGQGLEWMGIINPSGGSTSYAQKFQGRVTMTRDTSTSTVYMELSSLRSEDTAVYYCARDISGSYQTDAFDIWGQGTMVTVSSASTKGPSVFPLAPSSKSTSGGTAALGCLVKDYFPEPVTVSWNSGALTSGVHTFPAVLQSSGLYSLSSVVTVPSSSLGTQTYICNVNHKPSNTKVDKKVEPKSCDKTHTCPPCPAPELLGGPSVFLFPPKPKDTLMISRTPEVTCVVVDVSHEDPEVKFNWYVDGVEVHNAKTKPREEQYNSTYRVVSVLTVLHQDWLNGKEYKCKVSNKALPAPIEKTISKAKGQPREPQVYTLPPSRDELTKNQVSLTCLVKGFYPSDIAVEWESNGQPENNYKTTPPVLDSDGSFFLYSKLTVDKSRWQQGNVFSCSVMHEALHNHYTQKSLSLSPGK

SEQ ID NO: 203 - protein, 451 aa, synthetic construct
QVQLQDSGPGLVKPSQTLSLTCTVSGGSISSGGYYWSWIRQHPGKGLEWIGYIYYSGSTYYNPSLKSRVTISVDTSKNQFSLKLSSVTAADTAVYYCARVPVPLVGAFDIWGQGTMVTVSSASTKGPSVFPLAPSSKSTSGGTAALGCLVKDYFPEPVTVSWNSGALTSGVHTFPAVLQSSGLYSLSSVVTVPSSSLGTQTYICNVNHKPSNTKVDKKVEPKSCDKTHTCPPCPAPELLGGPSVFLFPPKPKDTLMISRTPEVTCVVVDVSHEDPEVKFNWYVDGVEVHNAKTKPREEQYNSTYRVVSVLTVLHQDWLNGKEYKCKVSNKALPAPIEKTISKAKGQPREPQVYTLPPSRDELTKNQVSLTCLVKGFYPSDIAVEWESNGQPENNYKTTPPVLDSDGSFFLYSKLTVDKSRWQQGNVFSCSVMHEALHNHYTQKSLSLSPGK

SEQ ID NO: 204 - protein, 449 aa, synthetic construct
RLQLQESGPGLVKPSQTLSLTCTVSGGSISSGGYYWSWIRQHPGKGLEWIGYIYYSGSTYYNPSLKSRVTISVDTSKNQFSLKLSSVTAADTAVYYCARATIYGYFDYWGQGTLVTVSSASTKGPSVFPLAPSSKSTSGGTAALGCLVKDYFPEPVTVSWNSGALTSGVHTFPAVLQSSGLYSLSSVVTVPSSSLGTQTYICNVNHKPSNTKVDKKVEPKSCDKTHTCPPCPAPELLGGPSVFLFPPKPKDTLMISRTPEVTCVVVDVSHEDPEVKFNWYVDGVEVHNAKTKPREEQYNSTYRVVSVLTVLHQDWLNGKEYKCKVSNKALPAPIEKTISKAKGQPREPQVYTLPPSRDELTKNQVSLTCLVKGFYPSDIAVEWESNGQPENNYKTTPPVLDSDGSFFLYSKLTVDKSRWQQGNVFSCSVMHEALHNHYTQKSLSLSPGK

SEQ ID NO: 205 - protein, 450 aa, synthetic construct
QVQLQESGPGLVKPSQTLSLTCTVSGGSISSGGYYWSWIRQHPGKGLEWIGYIYYSGSTYYNPSLKSRVTISVDTSKNQFSLKLSSVTAADTAVYYCARVRLLGGGFDIWGQGTTVTVSSASTKGPSVFPLAPSSKSTSGGTAALGCLVKDYFPEPVTVSWNSGALTSGVHTFPAVLQSSGLYSLSSVVTVPSSSLGTQTYICNVNHKPSNTKVDKKVEPKSCDKTHTCPPCPAPELLGGPSVFLFPPKPKDTLMISRTPEVTCVVVDVSHEDPEVKFNWYVDGVEVHNAKTKPREEQYNSTYRVVSVLTVLHQDWLNGKEYKCKVSNKALPAPIEKTISKAKGQPREPQVYTLPPSRDELTKNQVSLTCLVKGFYPSDIAVEWESNGQPENNYKTTPPVLDSDGSFFLYSKLTVDKSRWQQGNVFSCSVMHEALHNHYTQKSLSLSPGK

SEQ ID NO: 206 - protein, 454 aa, synthetic construct
EVQLVESGGGVVQPGRSLRLSCAASGFTFSSYAMHWVRQAPGKGLEWVAVISYDGSNKYYVDSVKGRFTISRDNSKNTLYLQMNSLRAEDTAVYYCARDRITYLDYYYYGMDVWGQGTTVTVSSASTKGPSVFPLAPSSKSTSGGTAALGCLVKDYFPEPVTVSWNSGALTSGVHTFPAVLQSSGLYSLSSVVTVPSSSLGTQTYICNVNHKPSNTKVDKKVEPKSCDKTHTCPPCPAPELLGGPSVFLFPPKPKDTLMISRTPEVTCVVVDVSHEDPEVKFNWYVDGVEVHNAKTKPREEQYNSTYRVVSVLTVLHQDWLNGKEYKCKVSNKALPAPIEKTISKAKGQPREPQVYTLPPSRDELTKNQVSLTCLVKGFYPSDIAVEWESNGQPENNYKTTPPVLDSDGSFFLYSKLTVDKSRWQQGNVFSCSVMHEALHNHYTQKSLSLSPGK

SEQ ID NO: 207 - protein, 450 aa, synthetic construct
QVQLQQSGPGLVKPSQTLSLTCAISGDSVSSDSAAWNWIRQSPSRGLEWLGRTYYRSKWYNDYAVSVKSRITINPDTSKNQFSLQLNSVTSDDTAVYYCARGSWAAPWLWGQGTLVTVSSASTKGPSVFPLAPSSKSTSGGTAALGCLVKDYFPEPVTVSWNSGALTSGVHTFPAVLQSSGLYSLSSVVTVPSSSLGTQTYICNVNHKPSNTKVDKKVEPKSCDKTHTCPPCPAPELLGGPSVFLFPPKPKDTLMISRTPEVTCVVVDVSHEDPEVKFNWYVDGVEVHNAKTKPREEQYNSTYRVVSVLTVLHQDWLNGKEYKCKVSNKALPAPIEKTISKAKGQPREPQVYTLPPSRDELTKNQVSLTCLVKGFYPSDIAVEWESNGQPENNYKTTPPVLDSDGSFFLYSKLTVDKSRWQQGNVFSCSVMHEALHNHYTQKSLSLSPGK

SEQ ID NO: 208 - protein, 447 aa, synthetic construct
QVQLLESGPGLVKPSQTVSLTCTVSGVSISRGVYSWSWIRQHPGKGLEWIGFIDYNGRTDYNPSLKSRVTISQDTSKNDFSLKLTSVTAADTAIYYCARGLHAFDIWGQGTMVTVSSASTKGPSVFPLAPSSKSTSGGTAALGCLVKDYFPEPVTVSWNSGALTSGVHTFPAVLQSSGLYSLSSVVTVPSSSLGTQTYICNVNHKPSNTKVDKKVEPKSCDKTHTCPPCPAPELLGGPSVFLFPPKPKDTLMISRTPEVTCVVVDVSHEDPEVKFNWYVDGVEVHNAKTKPREEQYNSTYRVVSVLTVLHQDWLNGKEYKCKVSNKALPAPIEKTISKAKGQPREPQVYTLPPSRDELTKNQVSLTCLVKGFYPSDIAVEWESNGQPENNYKTTPPVLDSDGSFFLYSKLTVDKSRWQQGNVFSCSVMHEALHNHYTQKSLSLSPGK

SEQ ID NO: 209 - protein, 450 aa, synthetic construct
RLQLQESGPRLVKPSETLSLTCSVSGGSISSRNHYWAWIRQPPGKGLEWIGYIYYSGSTYYNPSLKSRVTISVDTSKNQFSLKLSSVTAADTAVYYCARVGLLLRDFDYWGQGTLVTVSSASTKGPSVFPLAPSSKSTSGGTAALGCLVKDYFPEPVTVSWNSGALTSGVHTFPAVLQSSGLYSLSSVVTVPSSSLGTQTYICNVNHKPSNTKVDKKVEPKSCDKTHTCPPCPAPELLGGPSVFLFPPKPKDTLMISRTPEVTCVVVDVSHEDPEVKFNWYVDGVEVHNAKTKPREEQYNSTYRVVSVLTVLHQDWLNGKEYKCKVSNKALPAPIEKTISKAKGQPREPQVYTLPPSRDELTKNQVSLTCLVKGFYPSDIAVEWESNGQPENNYKTTPPVLDSDGSFFLYSKLTVDKSRWQQGNVFSCSVMHEALHNHYTQKSLSLSPGK

SEQ ID NO: 210 - protein, 452 aa, synthetic construct
EVQLVESGGGVVQPGRSLRLSCAASGFTFSSYAMHWVRQAPGKGLEWVAVISYDGSNKYYADSVKGRFTISRDNSKNTLYLQMNSLRAEDTAVYYCARDCSGGSCYDAFDIWGQGTMVTVSSASTKGPSVFPLAPSSKSTSGGTAALGCLVKDYFPEPVTVSWNSGALTSGVHTFPAVLQSSGLYSLSSVVTVPSSSLGTQTYICNVNHKPSNTKVDKKVEPKSCDKTHTCPPCPAPELLGGPSVFLFPPKPKDTLMISRTPEVTCVVVDVSHEDPEVKFNWYVDGVEVHNAKTKPREEQYNSTYRVVSVLTVLHQDWLNGKEYKCKVSNKALPAPIEKTISKAKGQPREPQVYTLPPSRDELTKNQVSLTCLVKGFYPSDIAVEWESNGQPENNYKTTPPVLDSDGSFFLYSKLTVDKSRWQQGNVFSCSVMHEALHNHYTQKSLSLSPGK

SEQ ID NO: 211 - protein, 451 aa, synthetic construct
QVQLQESGPGLVKPSQTLSLTCTVSGGSISSGGYYWSWIRQHPGKGLEWIGYIYYSGSTYYNPSLKSRVTISVDTSKNQFSLKLSSVTAADTAVYYCARVGVALHYGMDVWGQGTTVTVSSASTKGPSVFPLAPSSKSTSGGTAALGCLVKDYFPEPVTVSWNSGALTSGVHTFPAVLQSSGLYSLSSVVTVPSSSLGTQTYICNVNHKPSNTKVDKKVEPKSCDKTHTCPPCPAPELLGGPSVFLFPPKPKDTLMISRTPEVTCVVVDVSHEDPEVKFNWYVDGVEVHNAKTKPREEQYNSTYRVVSVLTVLHQDWLNGKEYKCKVSNKALPAPIEKTISKAKGQPREPQVYTLPPSRDELTKNQVSLTCLVKGFYPSDIAVEWESNGQPENNYKTTPPVLDSDGSFFLYSKLTVDKSRWQQGNVFSCSVMHEALHNHYTQKSLSLSPGK

SEQ ID NO: 212 - protein, 447 aa, synthetic construct
EVQLVESGGVVVQPGGSLRLSCAASGFTFDDYTMHWVRQAPGKGLEWVSLISWDGGSTYYADSVKGRFTISRDNAKNTLYLQMNSLRAEDTAVYYCARDTGYAMDVWGQGTMVTVSSASTKGPSVFPLAPSSKSTSGGTAALGCLVKDYFPEPVTVSWNSGALTSGVHTFPAVLQSSGLYSLSSVVTVPSSSLGTQTYICNVNHKPSNTKVDKKVEPKSCDKTHTCPPCPAPELLGGPSVFLFPPKPKDTLMISRTPEVTCVVVDVSHEDPEVKFNWYVDGVEVHNAKTKPREEQYNSTYRVVSVLTVLHQDWLNGKEYKCKVSNKALPAPIEKTISKAKGQPREPQVYTLPPSRDELTKNQVSLTCLVKGFYPSDIAVEWESNGQPENNYKTTPPVLDSDGSFFLYSKLTVDKSRWQQGNVFSCSVMHEALHNHYTQKSLSLSPGK

SEQ ID NO: 213 - protein, 450 aa, synthetic construct
QVQLVQSGAEVKKPGSSVKVSCKASGGTFSSYAISWVRQAPGQGLEWMGRIIPILGIANYAQKFQGRVTITADKSTSTAYMELSSLRSEDTAVYYCARAEGSSWYYFDYWGQGTLVTVSSASTKGPSVFPLAPSSKSTSGGTAALGCLVKDYFPEPVTVSWNSGALTSGVHTFPAVLQSSGLYSLSSVVTVPSSSLGTQTYICNVNHKPSNTKVDKKVEPKSCDKTHTCPPCPAPELLGGPSVFLFPPKPKDTLMISRTPEVTCVVVDVSHEDPEVKFNWYVDGVEVHNAKTKPREEQYNSTYRVVSVLTVLHQDWLNGKEYKCKVSNKALPAPIEKTISKAKGQPREPQVYTLPPSRDELTKNQVSLTCLVKGFYPSDIAVEWESNGQPENNYKTTPPVLDSDGSFFLYSKLTVDKSRWQQGNVFSCSVMHEALHNHYTQKSLSLSPGK

SEQ ID NO: 214 - protein, 450 aa, synthetic construct
QLQLQESGPGLVKPSGTLSLTCAVSGGSISSSNWWSWVRQPPGKGLEWIGEIYHSGSTNYNPSLKSRVTISVDKSKNQFSLKLSSVTAADTAVYYCARAHSRYYYGLDYWGQGTLVTVSSASTKGPSVFPLAPSSKSTSGGTAALGCLVKDYFPEPVTVSWNSGALTSGVHTFPAVLQSSGLYSLSSVVTVPSSSLGTQTYICNVNHKPSNTKVDKKVEPKSCDKTHTCPPCPAPELLGGPSVFLFPPKPKDTLMISRTPEVTCVVVDVSHEDPEVKFNWYVDGVEVHNAKTKPREEQYNSTYRVVSVLTVLHQDWLNGKEYKCKVSNKALPAPIEKTISKAKGQPREPQVYTLPPSRDELTKNQVSLTCLVKGFYPSDIAVEWESNGQPENNYKTTPPVLDSDGSFFLYSKLTVDKSRWQQGNVFSCSVMHEALHNHYTQKSLSLSPGK

SEQ ID NO: 215 - protein, 450 aa, synthetic construct
QVQLQQWGAELVKPGASVKLSCTASGFNIKDTYMHWVKQRPEQGLEWIGRIDPANGNTKYDPKFQGKATITADTSSNTAYLQLSSLTSEDTAVYYCARSYYRYDGYFDVWGAGTMVTVSSASTKGPSVFPLAPSSKSTSGGTAALGCLVKDYFPEPVTVSWNSGALTSGVHTFPAVLQSSGLYSLSSVVTVPSSSLGTQTYICNVNHKPSNTKVDKKVEPKSCDKTHTCPPCPAPELLGGPSVFLFPPKPKDTLMISRTPEVTCVVVDVSHEDPEVKFNWYVDGVEVHNAKTKPREEQYNSTYRVVSVLTVLHQDWLNGKEYKCKVSNKALPAPIEKTISKAKGQPREPQVYTLPPSRDELTKNQVSLTCLVKGFYPSDIAVEWESNGQPENNYKTTPPVLDSDGSFFLYSKLTVDKSRWQQGNVFSCSVMHEALHNHYTQKSLSLSPGK

SEQ ID NO: 216 - protein, 451 aa, synthetic construct
RLQLQESGPGLVKPSETLSLTCTVSGGSISSSSYYWGWIRQPPGKGLEWIGSIYYSGSTYYNPSLKSRVTISVDTSKNQFSLKLSSVTAADTAVYYCARRYSYGRDAFDIWGQGTMVTVSSASTKGPSVFPLAPSSKSTSGGTAALGCLVKDYFPEPVTVSWNSGALTSGVHTFPAVLQSSGLYSLSSVVTVPSSSLGTQTYICNVNHKPSNTKVDKKVEPKSCDKTHTCPPCPAPELLGGPSVFLFPPKPKDTLMISRTPEVTCVVVDVSHEDPEVKFNWYVDGVEVHNAKTKPREEQYNSTYRVVSVLTVLHQDWLNGKEYKCKVSNKALPAPIEKTISKAKGQPREPQVYTLPPSRDELTKNQVSLTCLVKGFYPSDIAVEWESNGQPENNYKTTPPVLDSDGSFFLYSKLTVDKSRWQQGNVFSCSVMHEALHNHYTQKSLSLSPGK

SEQ ID NO: 217 - protein, 449 aa, synthetic construct
QLQLQESGPGLVKPSETLSLTCTVSGGSISSSSYYWGWIRQPPGKGLEWIGSIYYSGSTYYNPSLKSRVTISVDTSKNQFSLKLSSVTAADTAVYYCARLTIFGVVLYWGQGTLVTVSSASTKGPSVFPLAPSSKSTSGGTAALGCLVKDYFPEPVTVSWNSGALTSGVHTFPAVLQSSGLYSLSSVVTVPSSSLGTQTYICNVNHKPSNTKVDKKVEPKSCDKTHTCPPCPAPELLGGPSVFLFPPKPKDTLMISRTPEVTCVVVDVSHEDPEVKFNWYVDGVEVHNAKTKPREEQYNSTYRVVSVLTVLHQDWLNGKEYKCKVSNKALPAPIEKTISKAKGQPREPQVYTLPPSRDELTKNQVSLTCLVKGFYPSDIAVEWESNGQPENNYKTTPPVLDSDGSFFLYSKLTVDKSRWQQGNVFSCSVMHEALHNHYTQKSLSLSPGK

SEQ ID NO: 218 - protein, 447 aa, synthetic construct
EVQLLESGGGVVQPGRSLRLSCAASGFTFSSYAMHWVRQAPGKGLEWVAVISYDGSNKYYADSVKGRFTISRDNSKNTLYLQMNSLRAEDTAVYYCARGKYNWFDPWGQGTLVTVSSASTKGPSVFPLAPSSKSTSGGTAALGCLVKDYFPEPVTVSWNSGALTSGVHTFPAVLQSSGLYSLSSVVTVPSSSLGTQTYICNVNHKPSNTKVDKKVEPKSCDKTHTCPPCPAPELLGGPSVFLFPPKPKDTLMISRTPEVTCVVVDVSHEDPEVKFNWYVDGVEVHNAKTKPREEQYNSTYRVVSVLTVLHQDWLNGKEYKCKVSNKALPAPIEKTISKAKGQPREPQVYTLPPSRDELTKNQVSLTCLVKGFYPSDIAVEWESNGQPENNYKTTPPVLDSDGSFFLYSKLTVDKSRWQQGNVFSCSVMHEALHNHYTQKSLSLSPGK

SEQ ID NO: 219 - protein, 448 aa, synthetic construct
QVQLVDSGGGLVQPGGSLRLSCVASGFAFSNYEMNWVRQAPGKGLEWVSYISSSSSYTNYADSVKGRFTISRDNAKNSLYLQMNSLRAEDTAVYYCARAQVRDAFDIWGQGTTVTVSSASTKGPSVFPLAPSSKSTSGGTAALGCLVKDYFPEPVTVSWNSGALTSGVHTFPAVLQSSGLYSLSSVVTVPSSSLGTQTYICNVNHKPSNTKVDKKVEPKSCDKTHTCPPCPAPELLGGPSVFLFPPKPKDTLMISRTPEVTCVVVDVSHEDPEVKFNWYVDGVEVHNAKTKPREEQYNSTYRVVSVLTVLHQDWLNGKEYKCKVSNKALPAPIEKTISKAKGQPREPQVYTLPPSRDELTKNQVSLTCLVKGFYPSDIAVEWESNGQPENNYKTTPPVLDSDGSFFLYSKLTVDKSRWQQGNVFSCSVMHEALHNHYTQKSLSLSPGK